European Patent Application EP 4 435 009 A2, published September 25, 2024. Title: CLAUDIN6 ANTIBODIES AND METHODS OF TREATING CANCER. Applicant: THE REGENTS OF THE UNIVERSITY OF CALIFORNIA. The sequence listing filed with the application follows.

SEQUENCE LISTING (489 sequences)

SEQ ID NO: 1 - protein, 220 aa, Homo sapiens
  REGION 1..220: note = NCBI / NP_067018.2, 2017-06-04
MASAGMQILGVVLTLLGWVNGLVSCALPMWKVTAFIGNSIVVAQVVWEGLWMSCVVQSTGQMQCKVYDSLLALPQDLQAARALCVIALLVALFGLLVYLAGAKCTTCVEEKDSKARLVLTSGIVFVISGVLTLIPVCWTAHAIIRDFYNPLVAEAQKRELGASLYLGWAASGLLLLGGGLLCCTCPSGGSQGPSHYMARYSTSAPAISRGPSEYPTKNYV

SEQ ID NO: 2 - protein, 23 aa, Homo sapiens
WTAHAIIRDFYNPLVAEAQKREL

SEQ ID NO: 3 - protein, 13 aa, Homo sapiens
TAHAIIRDFYNPL

SEQ ID NO: 4 - protein, 10 aa, Homo sapiens
LVAEAQKREL

SEQ ID NO: 5 - protein, 220 aa, Homo sapiens
  REGION 1..220: note = NCBI / NP_001297.1, 2017-07-10
MSMGLEITGTALAVLGWLGTIVCCALPMWRVSAFIGSNIITSQNIWEGLWMNCVVQSTGQMQCKVYDSLLALPQDLQAARALIVVAILLAAFGLLVALVGAQCTNCVQDDTAKAKITIVAGVLFLLAALLTLVPVSWSANTIIRDFYNPVVPEAQKREMGAGLYVGWAAAALQLLGGALLCCSCPPREKKYTATKVVYSAPRSTGPGASLGTGYDRKDYV

SEQ ID NO: 6 - protein, 209 aa, Homo sapiens
  REGION 1..209: note = NCBI / NP_001296.1, 2017-07-10
MASMGLQVMGIALAVLGWLAVMLCCALPMWRVTAFIGSNIVTSQTIWEGLWMNCVVQSTGQMQCKVYDSLLALPQDLQAARALVIISIIVAALGVLLSVVGGKCTNCLEDESAKAKTMIVAGVVFLLAGLMVIVPVSWTAHNIIQDFYNPLVASGQKREMGASLYVGWAASGLLLLGGGLLCCNCPPRTDKPYSAKYSAARSAAASNYV

SEQ ID NO: 7 - protein, 217 aa, Homo sapiens
  REGION 1..217: note = NCBI / NP_066192.1, 2017-04-15
MASTGLELLGMTLAVLGWLGTLVSCALPLWKVTAFIGNSIVVAQVVWEGLWMSCVVQSTGQMQCKVYDSLLALPQDLQAARALCVIALLLALLGLLVAITGAQCTTCVEDEGAKARIVLTAGVILLLAGILVLIPVCWTAHAIIQDFYNPLVAEALKRELGASLYLGWAAAALLMLGGGLLCCTCPPPQVERPRGPRLGYSIPSRSGASGLDKRDYV

SEQ ID NO: 8 - protein, 7 aa, synthetic construct
  REGION 1..7: note = Synthetic peptide
SSVSSTY

SEQ ID NO: 9 - skipped

SEQ ID NO: 10 - protein, 9 aa, synthetic construct
  REGION 1..9: note = Synthetic peptide
HQYHRSPLT

SEQ ID NO: 11 - protein, 8 aa, synthetic construct
  REGION 1..8: note = Synthetic peptide
GYTFTTYT

SEQ ID NO: 12 - protein, 8 aa, synthetic construct
  REGION 1..8: note = Synthetic peptide
INPSSGYT

SEQ ID NO: 13 - protein, 9 aa, synthetic construct
  REGION 1..9: note = Synthetic peptide
ANGDYYVAY

SEQ ID NO: 14 - protein, 6 aa, synthetic construct
  REGION 1..6: note = Synthetic peptide
ENIYSY

SEQ ID NO: 15 - skipped

SEQ ID NO: 16 - protein, 9 aa, synthetic construct
  REGION 1..9: note = Synthetic peptide
QHHYTVPWT

SEQ ID NO: 17 - protein, 8 aa, synthetic construct
  REGION 1..8: note = Synthetic peptide
GFTFSDYW

SEQ ID NO: 18 - protein, 10 aa, synthetic construct
  REGION 1..10: note = Synthetic peptide
IRLKSDNYAT

SEQ ID NO: 19 - protein, 8 aa, synthetic construct
  REGION 1..8: note = Synthetic peptide
NDGPPSGC

SEQ ID NO: 20 - protein, 6 aa, synthetic construct
  REGION 1..6: note = Synthetic peptide
ENIYSY

SEQ ID NO: 21 - skipped

SEQ ID NO: 22 - protein, 9 aa, synthetic construct
  REGION 1..9: note = Synthetic peptide
QHHYTVPWT

SEQ ID NO: 23 - protein, 8 aa, synthetic construct
  REGION 1..8: note = Synthetic peptide
GFTFSNYW

SEQ ID NO: 24 - protein, 10 aa, synthetic construct
  REGION 1..10: note = Synthetic peptide
IRLKSDNYAT

SEQ ID NO: 25 - protein, 8 aa, synthetic construct
  REGION 1..8: note = Synthetic peptide
NDGPPSGC

SEQ ID NO: 26 - protein, 11 aa, synthetic construct
  REGION 1..11: note = Synthetic peptide
QSLVHSDGNTY

SEQ ID NO: 27 - skipped

SEQ ID NO: 28 - protein, 9 aa, synthetic construct
  REGION 1..9: note = Synthetic peptide
SQSTHVPYT

SEQ ID NO: 29 - protein, 8 aa, synthetic construct
  REGION 1..8: note = Synthetic peptide
GYTFTSYT

SEQ ID NO: 30 - protein, 8 aa, synthetic construct
  REGION 1..8: note = Synthetic peptide
INPSSTYT

SEQ ID NO: 31 - protein, 10 aa, synthetic construct
  REGION 1..10: note = Synthetic peptide
SRGELGGFAY

SEQ ID NO: 32 - protein, 11 aa, synthetic construct
  REGION 1..11: note = Synthetic peptide
QSIVHSNGNTY

SEQ ID NO: 33 - skipped

SEQ ID NO: 34 - protein, 9 aa, synthetic construct
  REGION 1..9: note = Synthetic peptide
FQGSHVPFT

SEQ ID NO: 35 - protein, 8 aa, synthetic construct
  REGION 1..8: note = Synthetic peptide
GYIFTHYI

SEQ ID NO: 36 - protein, 8 aa, synthetic construct
  REGION 1..8: note = Synthetic peptide
INPYNDGT

SEQ ID NO: 37 - protein, 13 aa, synthetic construct
  REGION 1..13: note = Synthetic peptide
ARYYGYPYYSMDY

SEQ ID NO: 38 - protein, 12 aa, synthetic construct
  REGION 1..12: note = Synthetic peptide
QSLLNSRTRKNY

SEQ ID NO: 39 - skipped

SEQ ID NO: 40 - protein, 8 aa, synthetic construct
  REGION 1..8: note = Synthetic peptide
KQSYYLYT

SEQ ID NO: 41 - protein, 9 aa, synthetic construct
  REGION 1..9: note = Synthetic peptide
GYSITSGYY

SEQ ID NO: 42 - protein, 7 aa, synthetic construct
  REGION 1..7: note = Synthetic peptide
ISYDGGI

SEQ ID NO: 43 - protein, 10 aa, synthetic construct
  REGION 1..10: note = Synthetic peptide
ARFGKGAMDY

SEQ ID NO: 44 - protein, 7 aa, synthetic construct
  REGION 1..7: note = Synthetic peptide
SSVSSSY

SEQ ID NO: 45 - skipped

SEQ ID NO: 46 - protein, 9 aa, synthetic construct
  REGION 1..9: note = Synthetic peptide
HQYHRSPPT

SEQ ID NO: 47 - protein, 8 aa, synthetic construct
  REGION 1..8: note = Synthetic peptide
GYSFTGYT

SEQ ID NO: 48 - protein, 8 aa, synthetic construct
  REGION 1..8: note = Synthetic peptide
INPYNGGT

SEQ ID NO: 49 - protein, 12 aa, synthetic construct
  REGION 1..12: note = Synthetic peptide
ARGVYDYDGFTY

SEQ ID NO: 50 - protein, 11 aa, synthetic construct
  REGION 1..11: note = Synthetic peptide
QSLVHSDGNTY

SEQ ID NO: 51 - skipped

SEQ ID NO: 52 - protein, 9 aa, synthetic construct
  REGION 1..9: note = Synthetic peptide
SQSTHVPYT

SEQ ID NO: 53 - protein, 8 aa, synthetic construct
  REGION 1..8: note = Synthetic peptide
GYTFTTYT

SEQ ID NO: 54 - protein, 8 aa, synthetic construct
  REGION 1..8: note = Synthetic peptide
INPRSGYS

SEQ ID NO: 55 - protein, 10 aa, synthetic construct
  REGION 1..10: note = Synthetic peptide
SRGELGGFAY

SEQ ID NO: 56 - protein, 6 aa, synthetic construct
  REGION 1..6: note = Synthetic peptide
QTIGTW

SEQ ID NO: 57 - skipped

SEQ ID NO: 58 - protein, 9 aa, synthetic construct
  REGION 1..9: note = Synthetic peptide
QQLYSIPRT

SEQ ID NO: 59 - protein, 8 aa, synthetic construct
  REGION 1..8: note = Synthetic peptide
GYRFTDYN

SEQ ID NO: 60 - protein, 8 aa, synthetic construct
  REGION 1..8: note = Synthetic peptide
INPNNGGT

SEQ ID NO: 61 - protein, 10 aa, synthetic construct
  REGION 1..10: note = Synthetic peptide
ARDYLYFFDC

SEQ ID NO: 62 - protein, 11 aa, synthetic construct
  REGION 1..11: note = Synthetic peptide
QSLVHSNGNTY

SEQ ID NO: 63 - skipped

SEQ ID NO: 64 - protein, 9 aa, synthetic construct
  REGION 1..9: note = Synthetic peptide
SQITHVPYT

SEQ ID NO: 65 - protein, 8 aa, synthetic construct
  REGION 1..8: note = Synthetic peptide
GYTFTDYS

SEQ ID NO: 66 - protein, 8 aa, synthetic construct
  REGION 1..8: note = Synthetic peptide
ISTETGEP

SEQ ID NO: 67 - protein, 10 aa, synthetic construct
  REGION 1..10: note = Synthetic peptide
TRGLWSSFAY

SEQ ID NO: 68 - protein, 10 aa, synthetic construct
  REGION 1..10: note = Synthetic peptide
KSVSTSGYSY

SEQ ID NO: 69 - skipped

SEQ ID NO: 70 - protein, 9 aa, synthetic construct
  REGION 1..9: note = Synthetic peptide
QHSRELPLT

SEQ ID NO: 71 - protein, 8 aa, synthetic construct
  REGION 1..8: note = Synthetic peptide
GFTFSSFG

SEQ ID NO: 72 - protein, 8 aa, synthetic construct
  REGION 1..8: note = Synthetic peptide
ISSDSRTI

SEQ ID NO: 73 - protein, 11 aa, synthetic construct
  REGION 1..11: note = Synthetic peptide
ARDYGRTYEAY

SEQ ID NO: 74 - protein, 6 aa, synthetic construct
  REGION 1..6: note = Synthetic peptide
QDIGGN

SEQ ID NO: 75 - skipped

SEQ ID NO: 76 - protein, 9 aa, synthetic construct
  REGION 1..9: note = Synthetic peptide
LQRNAYPLT

SEQ ID NO: 77 - protein, 8 aa, synthetic construct
  REGION 1..8: note = Synthetic peptide
GFTFSSYA

SEQ ID NO: 78 - protein, 7 aa, synthetic construct
  REGION 1..7: note = Synthetic peptide
IRSGGTT

SEQ ID NO: 79 - protein, 12 aa, synthetic construct
  REGION 1..12: note = Synthetic peptide
AKVGGNPYPMDY

SEQ ID NO: 80 - protein, 7 aa, synthetic construct
  REGION 1..7: note = Synthetic peptide
SSISSNY

SEQ ID NO: 81 - skipped

SEQ ID NO: 82 - protein, 9 aa, synthetic construct
  REGION 1..9: note = Synthetic peptide
QQGSSIPLT

SEQ ID NO: 83 - protein, 8 aa, synthetic construct
  REGION 1..8: note = Synthetic peptide
GYAFSNYL

SEQ ID NO: 84 - protein, 8 aa, synthetic construct
  REGION 1..8: note = Synthetic peptide
INPGSGGT

SEQ ID NO: 85 - protein, 15 aa, synthetic construct
  REGION 1..15: note = Synthetic peptide
ARSYFGRSYPYTMDY

SEQ ID NO: 86 - protein, 10 aa, synthetic construct
  REGION 1..10: note = Synthetic peptide
QSVDYDGDNY

SEQ ID NO: 87 - skipped

SEQ ID NO: 88 - protein, 9 aa, synthetic construct
  REGION 1..9: note = Synthetic peptide
QQSNEDPFT

SEQ ID NO: 89 - protein, 8 aa, synthetic construct
  REGION 1..8: note = Synthetic peptide
GYTFTDYA

SEQ ID NO: 90 - protein, 8 aa, synthetic construct
  REGION 1..8: note = Synthetic peptide
ISTYSGNT

SEQ ID NO: 91 - protein, 13 aa, synthetic construct
  REGION 1..13: note = Synthetic peptide
ARRGDYSLYAMDY

SEQ ID NO: 92 - protein, 12 aa, synthetic construct
  REGION 1..12: note = Synthetic peptide
QSVLFSSNQKNY

SEQ ID NO: 93 - skipped

SEQ ID NO: 94 - protein, 8 aa, synthetic construct
  REGION 1..8: note = Synthetic peptide
HQYLSSRT

SEQ ID NO: 95 - protein, 8 aa, synthetic construct
  REGION 1..8: note = Synthetic peptide
GFTFSSFG

SEQ ID NO: 96 - protein, 8 aa, synthetic construct
  REGION 1..8: note = Synthetic peptide
ISSDSRTI

SEQ ID NO: 97 - protein, 11 aa, synthetic construct
  REGION 1..11: note = Synthetic peptide
ARDYGRTYEAY

SEQ ID NO: 98 - protein, 10 aa, synthetic construct
  REGION 1..10: note = Synthetic peptide
ESVDNYGISF

SEQ ID NO: 99 - skipped

SEQ ID NO: 100 - protein, 9 aa, synthetic construct
  REGION 1..9: note = Synthetic peptide
QQSKEVPLT

SEQ ID NO: 101 - protein, 8 aa, synthetic construct
  REGION 1..8: note = Synthetic peptide
GFPFSSSA

SEQ ID NO: 102 - protein, 7 aa, synthetic construct
  REGION 1..7: note = Synthetic peptide
INSDGNT

SEQ ID NO: 103 - protein, 13 aa, synthetic construct
  REGION 1..13: note = Synthetic peptide
TRNGDYRYDEFAY

SEQ ID NO: 104 - protein, 7 aa, synthetic construct
  REGION 1..7: note = Synthetic peptide
SSVSSSY

SEQ ID NO: 105 - skipped

SEQ ID NO: 106 - protein, 9 aa, synthetic construct
  REGION 1..9: note = Synthetic peptide
HQYHRSPPT

SEQ ID NO: 107 - protein, 8 aa, synthetic construct
  REGION 1..8: note = Synthetic peptide
GYTFTGYW

SEQ ID NO: 108 - protein, 8 aa, synthetic construct
  REGION 1..8: note = Synthetic peptide
INPSTGYT

SEQ ID NO: 109 - protein, 12 aa, synthetic construct
  REGION 1..12: note = Synthetic peptide
AREGITTVLVDY

SEQ ID NO: 110 - protein, 12 aa, synthetic construct
  REGION 1..12: note = Synthetic peptide
QSVLFSSNQKNY

SEQ ID NO: 111 - skipped

SEQ ID NO: 112 - protein, 8 aa, synthetic construct
  REGION 1..8: note = Synthetic peptide
HQYLSSRT

SEQ ID NO: 113 - protein, 8 aa, synthetic construct
  REGION 1..8: note = Synthetic peptide
GYSFTGYN

SEQ ID NO: 114 - protein, 8 aa, synthetic construct
  REGION 1..8: note = Synthetic peptide
IDPYYGGS

SEQ ID NO: 115 - protein, 14 aa, synthetic construct
  REGION 1..14: note = Synthetic peptide
ARERSGYVFSAMDY

SEQ ID NO: 116 - protein, 12 aa, synthetic construct
  REGION 1..12: note = Synthetic peptide
QSVLFSSNQKNY

SEQ ID NO: 117 - skipped

SEQ ID NO: 118 - protein, 8 aa, synthetic construct
  REGION 1..8: note = Synthetic peptide
HQYLSSRT

SEQ ID NO: 119 - protein, 8 aa, synthetic construct
  REGION 1..8: note = Synthetic peptide
GYSFTGYT

SEQ ID NO: 120 - protein, 8 aa, synthetic construct
  REGION 1..8: note = Synthetic peptide
INPYNGVT

SEQ ID NO: 121 - protein, 16 aa, synthetic construct
  REGION 1..16: note = Synthetic peptide
TRDPLYYGYRDSTMDY

SEQ ID NO: 122 - protein, 11 aa, synthetic construct
  REGION 1..11: note = Synthetic peptide
QSLVHSDGNTY

SEQ ID NO: 123 - skipped

SEQ ID NO: 124 - protein, 9 aa, synthetic construct
  REGION 1..9: note = Synthetic peptide
SQSTHVPYT

SEQ ID NO: 125 - protein, 8 aa, synthetic construct
  REGION 1..8: note = Synthetic peptide
GYTFTSYT

SEQ ID NO: 126 - protein, 8 aa, synthetic construct
  REGION 1..8: note = Synthetic peptide
INPSSTYT

SEQ ID NO: 127 - protein, 10 aa, synthetic construct
  REGION 1..10: note = Synthetic peptide
SRGELGGFAY

SEQ ID NO: 128 - protein, 6 aa, synthetic construct
  REGION 1..6: note = Synthetic peptide
QGIRGN

SEQ ID NO: 129 - skipped

SEQ ID NO: 130 - protein, 9 aa, synthetic construct
  REGION 1..9: note = Synthetic peptide
LQRNAYPLT

SEQ ID NO: 131 - protein, 8 aa, synthetic construct
  REGION 1..8: note = Synthetic peptide
GFTFSSFA

SEQ ID NO: 132 - protein, 7 aa, synthetic construct
  REGION 1..7: note = Synthetic peptide
IRSGGIT

SEQ ID NO: 133 - protein, 13 aa, synthetic construct
  REGION 1..13: note = Synthetic peptide
ARVSTATYYGMDY

SEQ ID NO: 134 - protein, 108 aa, synthetic construct
  REGION 1..108: note = Synthetic peptide
QIVLTQSPAIMSASLGERVTMTCTASSSVSSTYFHWYQQKPGSSPKLWIYSTSNLASGVPRRFSGSASGTSYSLTISSMEAEDAATYYCHQYHRSPLTFGAGTKLELK

SEQ ID NO: 135 - protein, 116 aa, synthetic construct
  REGION 1..116: note = Synthetic peptide
QVQLQQSAAELARPGASVKMSCKASGYTFTTYTMHWVKQRPGQGLEWIGFINPSSGYTDYNQKFKDRTTLTADKSSSTVYMQLSSLTSEDSAVYYCANGDYYVAYWGQGTLVTVSA

SEQ ID NO: 136 - protein, 107 aa, synthetic construct
  REGION 1..107: note = Synthetic peptide
DIQMTQSPASLSASVGETVTITCRISENIYSYLAWYQQKQGKSPQLLVYNAKILVEGVPSRFSGSGSGTQFSLKINSLQPEDFGNYYCQHHYTVPWTFGGGTKLEIK

SEQ ID NO: 137 - protein, 117 aa, synthetic construct
  REGION 1..117: note = Synthetic peptide
EVKLEESGGGLVQPGGSMKLSCVASGFTFSDYWMNWVRQSPEKGLEWVAQIRLKSDNYATHYAESVKGRFTISRDDSKRSVYLQMNNLRAEDTGTYYCNDGPPSGCWGQGTTLIVSS

SEQ ID NO: 138 - protein, 107 aa, synthetic construct; identical to SEQ ID NO: 136
  REGION 1..107: note = Synthetic peptide

SEQ ID NO: 139 - protein, 117 aa, synthetic construct
  REGION 1..117: note = Synthetic peptide
EVKLEESGGGLVQPGGSMKLSCVASGFTFSNYWMNWVRQSPEKGLEWVAQIRLKSDNYATHYAESVKGRFTISRDDSKRSVYLQMNNLRAEDTGTYYCNDGPPSGCWGQGTTLIVSS

SEQ ID NO: 140 - protein, 112 aa, synthetic construct
  REGION 1..112: note = Synthetic peptide
DVVMTQTPLSLPVSLGDQASISCRSSQSLVHSDGNTYLNWYLQKPGQSPKLLIYKVSNRFSGVPDRFSGSGSGTDFTLKIRRVEAEDLGVYFCSQSTHVPYTFGGGTKLEIK

SEQ ID NO: 141 - protein, 117 aa, synthetic construct
  REGION 1..117: note = Synthetic peptide
QVQLQQSGAELARPGASVKMSCKASGYTFTSYTMHWIKQRPGQGQEWIGYINPSSTYTHYIKKFKDKATLTADKSSSTAYMQLRSLTSEDSAVYYCSRGELGGFAYWGQGTLVTVSA

SEQ ID NO: 142 - protein, 112 aa, synthetic construct
  REGION 1..112: note = Synthetic peptide
DVLMTQTPLSLPVSLGDQPSISCRSSQSIVHSNGNTYLDWYLQKPGQSPKLLIYKVSNRFSGVPDRFSGSGSGTDFTLKISRVEAEDLGVYYCFQGSHVPFTFGSGTRLEIK

SEQ ID NO: 143 - protein, 120 aa, synthetic construct
  REGION 1..120: note = Synthetic peptide
EVQLQQSGPELVKPGASVKMSCKASGYIFTHYIMHWVKQKPGQGLEWIGCINPYNDGTKYNEKFKGKATLTSDKSSSTAYMELSSLTSEDSAVYYCARYYGYPYYSMDYWGQGTSVTVSS

SEQ ID NO: 144 - protein, 112 aa, synthetic construct
  REGION 1..112: note = Synthetic peptide
AIVMFQSPSSLVVSAGEKVTMSCKSSQSLLNSRTRKNYLAWYQQKPGQSPKLLIYWASTRESGVPDRFTGSGSGTDFTLTISSVQAEDLAVYYCKQSYYLYTFGGGTKLEIK

SEQ ID NO: 145 - protein, 117 aa, synthetic construct
  REGION 1..117: note = Synthetic peptide
DVQLQESGPGLVKSSQSLSLTCSVTGYSITSGYYWKWIRQFPGNKLEWMGYISYDGGINYNPSLKNRISITRDTSKNQFFLKLNSVTTEDTAKYYCARFGKGAMDYWGQGTSVTVSS

SEQ ID NO: 146 - protein, 108 aa, synthetic construct
  REGION 1..108: note = Synthetic peptide
QIVLTQSPAIMSASLGDRVTMTCTASSSVSSSYLHWYQQKPGSSPKLWIYSTSNLASGVPARFSGSGSGTSYSLTISSMEAEDAATYYCHQYHRSPPTFGSGTKLEIK

SEQ ID NO: 147 - protein, 119 aa, synthetic construct
  REGION 1..119: note = Synthetic peptide
EVQLQQSGPELVKPGASMKISCKASGYSFTGYTMNWVKQSHGKNLEWIGLINPYNGGTNYNQKFKGKATLTVDKSSSTAYMELLSLTSEDSAVYYCARGVYDYDGFTYWGQGTLVTVSA

SEQ ID NO: 148 - protein, 112 aa, synthetic construct
  REGION 1..112: note = Synthetic peptide
DVVMTQTPLSLPVSLGDQASISCRSSQSLVHSDGNTYLYWYLQKPGQSPKLLIYKVSNRFSGVPDRFSGSGSGTDFTLKISRVEAEDLGVYFCSQSTHVPYTFGGGTKLEIK

SEQ ID NO: 149 - protein, 117 aa, synthetic construct
  REGION 1..117: note = Synthetic peptide
QVQLQQSGAELARPGASVKMSCKASGYTFTTYTMHWLKQRPGQGLEWIGYINPRSGYSNYNQKFKDKATLTADKSSNTAYMQLNTLTSEDSKVYYCSRGELGGFAYWGQGTLVTVSA

SEQ ID NO: 150 - protein, 107 aa, synthetic construct
  REGION 1..107: note = Synthetic peptide
DIQMTQSPASQSASLGESVTITCLASQTIGTWLAWYQQKPGKSPQLLIYAAASLADGVPSRFSGSGSGTRFSFKISSLQAEDFVSYYCQQLYSIPRTFGGGTKLEIK

SEQ ID NO: 151 - protein, 117 aa, synthetic construct
  REGION 1..117: note = Synthetic peptide
EVQLQQSGPELVKPGASVKMSCKASGYRFTDYNMHWVKQSHGKSLEWIGYINPNNGGTNYNQNFKGKATLTVNKSSSTAYMELRSLTSEDSAAYYCARDYLYFFDCWGQGTTLTVSS

SEQ ID NO: 152 - protein, 112 aa, synthetic construct
  REGION 1..112: note = Synthetic peptide
DVVMTQTPLSLPVSLGDQASISCRASQSLVHSNGNTYLHWFLQKPGQSPKLLIYKVSNRFSGVPDRFSGSGSRTDFTLKISRVEAEDLGVYFCSQITHVPYTFGGGTKLEIK

SEQ ID NO: 153 - protein, 117 aa, synthetic construct
  REGION 1..117: note = Synthetic peptide
QIQLVQSGPALKKPGETVKISCKASGYTFTDYSMHWIKQAPGKGLKWMGWISTETGEPTYADGFKGRFDFSLETSADTAYLSINNLTNEDTATYFCTRGLWSSFAYWGQGTLVTVSA

SEQ ID NO: 154 - protein, 111 aa, synthetic construct
  REGION 1..111: note = Synthetic peptide
DIVLTQSPASLAVSLGQRATISCRASKSVSTSGYSYIHWYQQKPGQPPKLLIYLASNLESGVPARFSGSGSGTDFTLNIHPVEEEDAATYYCQHSRELPLTFGAGTKLELK

SEQ ID NO: 155 - protein, 118 aa, synthetic construct
  REGION 1..118: note = Synthetic peptide
DVQLVESGGGLVQPRGSRKLSCAASGFTFSSFGMHWVRQAPEKGLEWVAYISSDSRTIYYADTVKGRFTISRDNPTNTLFLQMTSLRSEDTAMYYCARDYGRTYEAYWGQGTLVTVSA

SEQ ID NO: 156 - protein, 107 aa, synthetic construct
  REGION 1..107: note = Synthetic peptide
DIQMIQSPSSMFASLGDRVSLSCRASQDIGGNLDWYQQKPGGTIKLLIYSTSNLNSGVPSRFSGSGSGSDYSLTITSLESEDFADYYCLQRNAYPLTFGAGTKLELK

SEQ ID NO: 157 - protein, 118 aa, synthetic construct
  REGION 1..118: note = Synthetic peptide
EVKLMESGGDLVKPGGSLKLSCAASGFTFSSYAMSWVRQTPEKRLEWVASIRSGGTTYYPDSVKGRFTISRDNARNILYLRMSSLRSEDTAIYYCAKVGGNPYPMDYWGQGTSVTVSS

SEQ ID NO: 158 - protein, 108 aa, synthetic construct
  REGION 1..108: note = Synthetic peptide
EIVLTQSPTTMAASPGEKITITCSASSSISSNYLHWYQQKPGFSPKLLIYRTSNLASGVPARFSGSGSGTSYSLTIGTMEAEDVATYYCQQGSSIPLTFGAGTKLELK

SEQ ID NO: 159 - protein, 122 aa, synthetic construct
  REGION 1..122: note = Synthetic peptide
QVQLQQSGAELVRPGTSVKVSCKASGYAFSNYLIEWVKQRPGQGLEWIGVINPGSGGTNYNEKFKGKATMTADKSSSTAYMHLSNLTSEDSVVYFCARSYFGRSYPYTMDYWGQGTSVTVSS

SEQ ID NO: 160 - protein, 111 aa, synthetic construct
  REGION 1..111: note = Synthetic peptide
DIVLTQSPASLAVSLGQRATISCKASQSVDYDGDNYVNWYQQKVGQPPKLLISAASNLESGIPARFSGSGSGTDFTLNIHPVEEEDAATYYCQQSNEDPFTFGSGTKLEIK

SEQ ID NO: 161 - protein, 120 aa, synthetic construct
  REGION 1..120: note = Synthetic peptide
QVQLQQSGPELVRPGVSVKISCKGSGYTFTDYAMHWVKQSHAKSLEWIGVISTYSGNTNYNQKFQDKATMTVDKSSSTAYMALARLTSDDSAIYYCARRGDYSLYAMDYWGQGTSVTVSS

SEQ ID NO: 162 - protein, 112 aa, synthetic construct
  REGION 1..112: note = Synthetic peptide
NIMMTQSPSSLAVSAGEKVTMSCKSSQSVLFSSNQKNYLAWYQQKPGQSPRLLIYWASTRESGVPDRFTGSGSGTDFTLTISNVQAEDLAVYYCHQYLSSRTFGAGTKLELK

SEQ ID NO: 163 - protein, 118 aa, synthetic construct; identical to SEQ ID NO: 155
  REGION 1..118: note = Synthetic peptide

SEQ ID NO: 164 - protein, 111 aa, synthetic construct
  REGION 1..111: note = Synthetic peptide
DIVLTQSPASLALSLGQRATISCRASESVDNYGISFMNWFQQKPGQPPKLLIYAASNQGSGVPARFSGSGSGTDFSLNIHPMEEDDTAMYFCQQSKEVPLTFGAGTKLELK

SEQ ID NO: 165 - protein, 119 aa, synthetic construct
  REGION 1..119: note = Synthetic peptide
EVRLVESGGGLMQPGGSLKLPCAASGFPFSSSAMSWVRQTPEKRLEWVASINSDGNTYYPDSVKGRFTISRDSARNILYLQMSSLRSEDTAMYYCTRNGDYRYDEFAYWGQGTLVTVSA

SEQ ID NO: 166 - protein, 108 aa, synthetic construct
  REGION 1..108: note = Synthetic peptide
QIVLTQSPAIMSASLGERVTMTCTASSSVSSSYLHWYQQKPGSSPKLWIYSTSNLASGVPARFSGSGSGTSYSLTISSMEAEDAATYYCHQYHRSPPTFGAGTKLELK

SEQ ID NO: 167 - protein, 119 aa, synthetic construct
  REGION 1..119: note = Synthetic peptide
QVQLQQSGAELAKPGASVKMSCKASGYTFTGYWMHWVKQRPGQGLEWLGYINPSTGYTESNQKFKDKATLTADKSSTTAYMQLRSLTPEDSAVYYCAREGITTVLVDYWGQGTTLTVSS

SEQ ID NO: 168 - protein, 112 aa, synthetic construct; identical to SEQ ID NO: 162
  REGION 1..112: note = Synthetic peptide

SEQ ID NO: 169 - protein, 121 aa, synthetic construct
  REGION 1..121: note = Synthetic peptide
QVQLKQSGPELEKPGASVKISCKASGYSFTGYNMNWVKQSNGKSLEWIGNIDPYYGGSTYNQKFTGKATLTVDKSSSTAYMQLKSLTSEDSAVYYCARERSGYVFSAMDYWGQGTSVTVSS

SEQ ID NO: 170 - protein, 112 aa, synthetic construct; identical to SEQ ID NO: 162
  REGION 1..112: note = Synthetic peptide

SEQ ID NO: 171 - protein, 123 aa, synthetic construct
  REGION 1..123: note = Synthetic peptide
EVQLQQSGPELVKPGGSMKISCKASGYSFTGYTMNWVKRSHGKNLEWIGLINPYNGVTTYNQNFKGKATLAVDKSSSTAYMELLGLTSEDSAVYYCTRDPLYYGYRDSTMDYWGQGTSVTVSS

SEQ ID NO: 172 - protein, 112 aa, synthetic construct; identical to SEQ ID NO: 140
  REGION 1..112: note = Synthetic peptide

SEQ ID NO: 173 - protein, 117 aa, synthetic construct
  REGION 1..117: note = Synthetic peptide
EVQLQQSGAELARPGASVKMSCKASGYTFTSYTMHWIKQRPGQGQEWIGYINPSSTYTHYIKKFKDKATLTADKSSSTAYMQLRSLTSEDSAVYYCSRGELGGFAYWGQGTLVTVSA

SEQ ID NO: 174 - protein, 107 aa, synthetic construct
  REGION 1..107: note = Synthetic peptide
DIQMIQSPSSMFASLGDRVSLSCRASQGIRGNLDWYQQKPGGTIKLLIYSTSILNSGVPSRFSGSGSGSDYSLTITSLESEDFADYYCLQRNAYPLTFGSGTKLELK

SEQ ID NO: 175 - protein, 119 aa, synthetic construct
  REGION 1..119: note = Synthetic peptide
EVKLVESGGGLMKPGGSLKLSCAASGFTFSSFALSWVRQTPEKRLEWVASIRSGGITYHADSVKGRFTISRDNAGNILYLQMNSLRSEDTAMYFCARVSTATYYGMDYWGQGTSVTVSS

SEQ ID NO: 176 - protein, 219 aa, Mus musculus
  REGION 1..219: note = NCBI / NP_061247.1, 2017-08-07
MASTGLQILGIVLTLLGWVNALVSCALPMWKVTAFIGNSIVVAQMVWEGLWMSCVVQSTGQMQCKVYDSLLALPQDLQAARALCVVTLLIVLLGLLVYLAGAKCTTCVEDRNSKSRLVLISGIIFVISGVLTLIPVCWTAHSIIQDFYNPLVADAQKRELGASLYLGWAASGLLLLGGGLLCCACSSGGTQGPRHYMACYSTSVPHSRGPSEYPTKNYV

SEQ ID NO: 177 - protein, 80 aa, synthetic construct
  REGION 1..80: note = Synthetic peptide
MASAGMQILGVVLTLLGWVNGLVSCALPMWKVTAFIGNSIVVAQVVWEGLWMSCVVQSTGQMQCKVYDSLLALPQDLQAA

SEQ ID NO: 178 - protein, 220 aa, synthetic construct
  REGION 1..220: note = Synthetic peptide
MASAGMQILGVVLTLLGWVNGLVSCALPMWKVTAFIGNSIVVAQVVWEGLWMSCVVQSTGQMQCKVYDSLLALPQDLQAARALCVIALLVALFGLLVYLAGAKCTTCVEEKDSKARLVLTSGIVFVISGVLTLIPVCWTAHAVIRDFYNPLVAEAQKRELGASLYLGWAASGLLLLGGGLLCCTCPSGGSQGPSHYMARYSTSAPAISRGPSEYPTKNYV

SEQ ID NO: 179 - protein, 322 aa, synthetic construct
  REGION 1..322: note = Synthetic peptide
CAGATCGTGCTGACTCAGAGTCCTTCAATTATGTCCGTGAGCCCAGGCGAGAAGGTCACCATCACATGCAGTGCCTCCAGCTCTGTCTCATACATGCACTGGTTCCAGCAGAAGCCAGGGACCAGTCCCAAGCTGTGCATCTACTCTACATCGAACCTGGCCTCCGGAGTGCCCGCAAGGTTTAGCGGTCGGGGCTCTGGAACTTCATACTCCCTGACCATCTCGCGGGTGGCCGCTGAGGATGCAGCAACATACTATTGCCAGCAGAGGTCCAATTATCCCCCTTGGACATTCGGCGGAGGTACCAAACTCGAGATTAAGC

SEQ ID NO: 180 - protein, 351 aa, synthetic construct
  REGION 1..351: note = Synthetic peptide
GAAGTCCAGCTGCAGCAGTCTGGCCCTGAACTGGTGAAGCCTGGCGCCAGCATGAAGATCTCCTGCAAGGCCAGCGGCTACTCCTTCACCGGCTATACAATGAACTGGGTGAAGCAGTCCCACGGCAAGAATCTGGAGTGGATCGGCCTGATCAACCCATACAATGGCGGCACCATCTACAACCAGAAGTTTAAGGGCAAGGCCACCCTGACAGTGGACAAGAGCTCCTCTACCGCCTACATGGAGCTGCTGTCTCTGACAAGCGAGGACTCCGCCGTGTACTATTGCGCCCGGGACTACGGCTTCGTGCTGGACTATTGGGGCCAGGGCACCACACTGACAGTGAGCTCC

SEQ ID NO: 181 - protein, 107 aa, synthetic construct
  REGION 1..107: note = Synthetic peptide
QIVLTQSPSIMSVSPGEKVTITCSASSSVSYMHWFQQKPGTSPKLCIYSTSNLASGVPARFSGRGSGTSYSLTISRVAAEDAATYYCQQRSNYPPWTFGGGTKLEIK

SEQ ID NO: 182 - protein, 117 aa, synthetic construct
  REGION 1..117: note = Synthetic peptide
EVQLQQSGPELVKPGASMKISCKASGYSFTGYTMNWVKQSHGKNLEWIGLINPYNGGTIYNQKFKGKATLTVDKSSSTAYMELLSLTSEDSAVYYCARDYGFVLDYWGQGTTLTVSS

SEQ ID NO: 183 - DNA, 324 bp, synthetic construct
  misc_feature 1..324: note = Synthetic polynucleotide
  source 1..324: mol_type = other DNA
gaaattgtgctcacccagtctccagcactcatggctgcatctccaggggagaaggtcaccatcacctgcagtgtcagctcaagtataagttccagcaacttgcactggtaccagcagaagtcaggaacctcccccaaactctggatttatggcacatccaacctggcttctggagtccctgttcgcttcagtggcagtggatctgggacctcttattctctcacaatcagcaacatggaggctgaagatgctgccacttattactgtcaacagtggagtagttacccacacacgttcggaggggggaccaagctggaaataaaa

SEQ ID NO: 184 - DNA, 378 bp, synthetic construct
  misc_feature 1..378: note = Synthetic polynucleotide
  source 1..378: mol_type = other DNA
caggtccaaatgcagcagtctggagctgagctggtaaggcctgggacttcagtgaaggtgtcctgcaaggcttctggatacgccttcactaattacttgatagagtgggtaaagcagaggcctggacagggccttgagtggattggactgattaatcctggaagtggtggtactaattacaatgagaagttcaagggcaaggcaacactgactgcagacaaatcctccaccactgcctacatgcagctcagcagcctgacatctgatgactctgcggtttatttctgtgcaagacggtcccctctagggagttggatctactatgcttacgacggtgttgcttactggggccaagggactctggtcactgtctctgca

SEQ ID NO: 185 - protein, 108 aa, synthetic construct
  REGION 1..108: note = Synthetic peptide
EIVLTQSPALMAASPGEKVTITCSVSSSISSSNLHWYQQKSGTSPKLWIYGTSNLASGVPVRFSGSGSGTSYSLTISNMEAEDAATYYCQQWSSYPHTFGGGTKLEIK

SEQ ID NO: 186 - protein, 126 aa, synthetic construct
  REGION 1..126: note = Synthetic peptide
QVQMQQSGAELVRPGTSVKVSCKASGYAFTNYLIEWVKQRPGQGLEWIGLINPGSGGTNYNEKFKGKATLTADKSSTTAYMQLSSLTSDDSAVYFCARRSPLGSWIYYAYDGVAYWGQGTLVTVSA

SEQ ID NO: 187 - DNA, 645 bp, Mus musculus
  source 1..645: mol_type = genomic DNA
gatattgtgctaactcagtctccagccaccctgtctgtgactccaggaaatagcgtcagtctttcctgcagggccagccaaagtattggcggtaacctacactggtatcaacaaaaatcacatgagtctccaaggcttctcatcaagtatgcttcccagtccatctctgggatcccctccaggttcagtggcagtggatcagggacagatttcactctcagtatcaacagtgtggagactgaagattttggaatgtatttctgtcaacagagtaacagctggccttacacgttcggaggggggaccaagctggaaataaaacgggcagatgctgcaccaactgtatccatcttcccaccatccagtgagcagttaacatctggaggtgcctcagtcgtgtgcttcttgaacaacttctaccccaaagacatcaatgtcaagtggaagattgatggcagtgaacgacaaaatggcgtcctgaacagttggactgatcaggacagcaaagacagcacctacagcatgagcagcaccctcacgttgaccaaggacgagtatgaacgacataacagctatacctgtgaggccactcacaagacatcaacttcacccattgtcaagagcttcaacaggaatgagtgttag

SEQ ID NO: 188 - DNA, 1335 bp, Mus musculus
  source 1..1335: mol_type = genomic DNA
gacgtgcagcttcaggagtcaggacctagcctcgtgaaaccttctcagactctgtccctcacctgttctgtcactggcgactccatcaccagtgattactggagctggatccggaaattcccagggaatagacttgagtacatggggtacgtaagctacagtggtagcacttactacaatccatctctcaaaagtcgaatctccatcacccgagacacatccaagaaccagtactacctggatttgaattctgtgactactgaggacacagccacatattactgtgcaaactgggacggtgattactggggccaagggactctggtcactgtctcttcagcagctaaaacaacagccccatcggtctatccactggcccctgtgtgtggagatacaactggctcctcggtgactctaggatgcctggtcaagggttatttccctgagccagtgaccttgacctggaactctggatccctgtccagtggtgtgcacaccttcccagctgtcctgcagtctgacctctacaccctcagcagctcagtgactgtaacctcgagcacctggcccagccagtccatcacctgcaatgtggcccacccggcaagcagcaccaaggtggacaagaaaattgagcccagagggcccacaatcaagccctgtcctccatgcaaatgcccagcacctaacctcttgggtggaccatccgtcttcatcttccctccaaagatcaaggatgtactcatgatctccctgagccccatagtcacatgtgtggtggtggatgtgagcgaggatgacccagatgtccagatcagctggtttgtgaacaacgtggaagtacacacagctcagacacaaacccatagagaggattacaacagtactctccgggtggtcagtgccctccccatccagcaccaggactggatgagtggcaaggagttcaaatgcaaggtcaacaacaaagacctcccagcgcccatcgagagaaccatctcaaaacccaaagggtcagtaagagctccacaggtatatgtcttgcctccaccagaagaagagatgactaagaaacaggtcactctgacctgcatggtcacagacttcatgcctgaagacatttacgtggagtggaccaacaacgggaaaacagagctaaactacaagaacactgaaccagtcctggactctgatggttcttacttcatgtacagcaagctgagagtggaaaagaagaactgggtggaaagaaatagctactcctgttcagtggtccacgagggtctgcacaatcaccacacgactaagagcttctcccggactccgggtaaatga

SEQ ID NO: 189 - DNA, 8806 bp, synthetic construct
  misc_feature 1..8806: note = Synthetic peptide
  source 1..8806: mol_type = other DNA
aatgtagtcttatgcaatactcttgtagtcttgcaacatggtaacgatgagttagcaacatgccttacaaggagagaaaaagcaccgtgcatgccgattggtggaagtaaggtggtacgatcgtgccttattaggaaggcaacagacgggtctgacatggattggacgaaccactgaattgccgcattgcagagatattgtatttaagtgcctagctcgatacataaacgggtctctctggttagaccagatctgagcctgggagctctctggctaactagggaacccactgcttaagcctcaataaagcttgccttgagtgcttcaagtagtgtgtgcccgtctgttgtgtgactctggtaactagagatccctcagacccttttagtcagtgtggaaaatctctagcagtggcgcccgaacagggacttgaaagcgaaagggaaaccagaggagctctctcgacgcaggactcggcttgctgaagcgcgcacggcaagaggcgaggggcggcgactggtgagtacgccaaaaattttgactagcggaggctagaaggagagagatgggtgcgagagcgtcagtattaagcgggggagaattagatcgcgatgggaaaaaattcggttaaggccagggggaaagaaaaaatataaattaaaacatatagtatgggcaagcagggagctagaacgattcgcagttaatcctggcctgttagaaacatcagaaggctgtagacaaatactgggacagctacaaccatcccttcagacaggatcagaagaacttagatcattatataatacagtagcaaccctctattgtgtgcatcaaaggatagagataaaagacaccaaggaagctttagacaagatagaggaagagcaaaacaaaagtaagaccaccgcacagcaagcggccgctgatcttcagacctggaggaggagatatgagggacaattggagaagtgaattatataaatataaagtagtaaaaattgaaccattaggagtagcacccaccaaggcaaagagaagagtggtgcagagagaaaaaagagcagtgggaataggagctttgttccttgggttcttgggagcagcaggaagcactatgggcgcagcgtcaatgacgctgacggtacaggccagacaattattgtctggtatagtgcagcagcagaacaatttgctgagggctattgaggcgcaacagcatctgttgcaactcacagtctggggcatcaagcagctccaggcaagaatcctggctgtggaaagatacctaaaggatcaacagctcctggggatttggggttgctctggaaaactcatttgcaccactgctgtgccttggaatgctagttggagtaataaatctctggaacagatttggaatcacacgacctggatggagtgggacagagaaattaacaattacacaagcttaatacactccttaattgaagaatcgcaaaaccagcaagaaaagaatgaacaagaattattggaattagataaatgggcaagtttgtggaattggtttaacataacaaattggctgtggtatataaaattattcataatgatagtaggaggcttggtaggtttaagaatagtttttgctgtactttctatagtgaatagagttaggcagggatattcaccattatcgtttcagacccacctcccaaccccgaggggacccgacaggcccgaaggaatagaagaagaaggtggagagagagacagagacagatccattcgattagtgaacggatctcgacggtatcggttaacttttaaaagaaaaggggggattggggggtacagtgcaggggaaagaatagtagacataatagcaacagacatacaaactaaagaattacaaaaacaaattacaaaaattcaaaattttccgataagcttgggagttccgcgttacataacttacggtaaatggcccgcctggctgaccgcccaacgacccccgcccattgacgtcaataatgacgtatgttcccatagtaacgccaatagggactttccattgacgtcaatgggtggagtatttacggtaaactgcccacttggcagtacatcaagtgtatcatatgccaagtacgccccctattgacgtcaatgacggtaaatggcccgcctggcattatgcccagtacatgaccttatgggactttcctacttggcagtacatctacgtattagtcatcgctattaccatggtgatgcggttttggcagtacatcaatgggcgtggatagcggtttgactcacggggatttccaagtctccaccccattgacgtcaatgggagtttgttttggcaccaaaatcaacgggactttccaaaatgtcgtaacaactccgccccattgacgcaaatgggcggtaggcgtgtacggtgggaggtctatataagcagagctcgtttagtgaaccgtcagatcgcctggagacgccatccacgctgttttgacctccatagaagacaccgactctagaactagtggatcccccgggctgcaggaattcgtcgactggatccggtaccgaggagatctgccgccgcgatcgccggcgcgccagatctcaagcttaactagttagcggaccgacgcgtacgcggccgctcgagatgagcgggggcgaggagctgttcgccggcatcgtgcccgtgctgatcgagctggacggcgacgtgcacggccacaagttcagcgtgcgcggcgagggcgagggcgacgccgactacggcaagctggagatcaagttcatctgcaccaccggcaagctgcccgtgccctggcccaccctggtgaccaccctctgctacggcatccagtgcttcgcccgctaccccgagcacatgaagatgaacgacttcttcaagagcgccatgcccgagggctacatccaggagcgcaccatccagttccaggacgacggcaagtacaagacccgcggcgaggtgaagttcgagggcgacaccctggtgaaccgcatcgagctgaagggcaaggacttcaaggaggacggcaacatcctgggccacaagctggagtacagcttcaacagccacaacgtgtacatccgccccgacaaggccaacaacggcctggaggctaacttcaagacccgccacaacatcgagggcggcggcgtgcagctggccgaccactaccagaccaacgtgcccctgggcgacggccccgtgctgatccccatcaaccactacctgagcactcagaccaagatcagcaaggaccgcaacgaggcccgcgaccacatggtgctcctggagtccttcagcgcctgctgccacacccacggcatggacgagctgtacaggtccggactcagataagtttaaacccgatatcatcatctagggcggccaattccgcccctctccccccccctaacgttactggccgaagccgcttggaataaggccggtgtgcgtttgtctatatgttattttccaccatattgccgtcttttggcaatgtgagggcccggaaacctggccctgtcttcttgacgagcattcctaggggtctttcccctctcgccaaaggaatgcaaggtctgttgaatgtcgtgaaggaagcagttcctctggaagcttcttgaagacaaacaacgtctgtagcgaccctttgcaggcagcggaaccccccacctggcgacaggtgcctctgcggccaaaagccacgtgtataagatacacctgcaaaggcggcacaaccccagtgccacgttgtgagttggatagttgtggaaagagtcaaatggctctcctcaagcgtattcaacaaggggctgaaggatgcccagaaggtaccccattgtatgggatctgatctggggcctcggtgcacatgctttacatgtgtttagtcgaggttaaaaaaacgtctaggccccccgaaccacggggacgtggttttcctttgaaaaacacgatgataagcttgccacaacccacaaggagacgaccttccatgaccgagtacaagcccacggtgcgcctcgccacccgcgacgacgtcccccgggccgtacgcaccctcgccgccgcgttcgccgactaccccgccacgcgccacaccgtcgacccggaccgccacatcgagcgggtcaccgagctgcaagaactcttcctcacgcgcgtcgggctcgacatcggcaaggtgtgggtcgcggacgacggcgccgcggtggcggtctggaccacgccggagagcgtcgaagcgggggcggtgttcgccgagatcggcccgcgcatggccgagttgagcggttcccggctggccgcgcagcaacagatggaaggcctcctggcgccgcaccggcccaaggagcccgcgtggttcctggccaccgtcggcgtctcgcccgaccaccagggcaagggtctgggcagcgccgtcgtgctccccggagtggaggcggccgagcgcgccggggtgcccgccttcctggagacctccgcgccccgcaacctccccttctacgagcggctcggcttcaccgtcaccgccgacgtcgaggtgcccgaaggaccgcgcacctggtgcatgacccgcaagcccggtgcctgaaattagatcgataccgtcgacaatcaacctctggattacaaaatttgtgaaagattgactggtattcttaactatgttgctccttttacgctatgtggatacgctgctttaatgcctttgtatcatgctattgcttcccgtatggctttcattttctcctccttgtataaatcctggttgctgtctctttatgaggagttgtggcccgttgtcaggcaacgtggcgtggtgtgcactgtgtttgctgacgcaacccccactggttggggcattgccaccacctgtcagctcctttccgggactttcgctttccccctccctattgccacggcggaactcatcgccgcctgccttgcccgctgctggacaggggctcggctgttgggcactgacaattccgtggtgttgtcggggaagctgacgtcctttccatggctgctcgcctgtgttgccacctggattctgcgcgggacgtccttctgctacgtcccttcggccctcaatccagcggaccttccttcccgcggcctgctgccggctctgcggcctcttccgcgtcttcgccttcgccctcagacgagtcggatctccctttgggccgcctccccgcctgaatacgagctcggtacctttaagaccaatgacttacaaggcagctgtagatcttagccactttttaaaagaaaaggggggactggaagggctaattcactcccaacgaagacaagatctgctttttgcttgtactgggtctctctggttagaccagatctgagcctgggagctctctggctaactagggaacccactgcttaagcctcaataaagcttgccttgagtgcttcaagtagtgtgtgcccgtctgttgtgtgactctggtaactagagatccctcagacccttttagtcagtgtggaaaatctctagcagtagtagttcatgtcatcttattattcagtatttataacttgcaaagaaatgaatatcagagagtgagaggaacttgtttattgcagcttataatggttacaaataaagcaatagcatcacaaatttcacaaataaagcatttttttcactgcattctagttgtggtttgtccaaactcatcaatgtatcttatcatgtctggctctagctatcccgcccctaactccgcccatcccgcccctaactccgcccagttccgcccattctccgccccatggctgactaattttttttatttatgcagaggccgaggccgcctcggcctctgagctattccagaagtagtgaggaggcttttttggaggcctagggacgtacccaattcgccctatagtgagtcgtattacgcgcgctcactggccgtcgttttacaacgtcgtgactgggaaaaccctggcgttacccaacttaatcgccttgcagcacatccccctttcgccagctggcgtaatagcgaagaggcccgcaccgatcgcccttcccaacagttgcgcagcctgaatggcgaatgggacgcgccctgtagcggcgcattaagcgcggcgggtgtggtggttacgcgcagcgtgaccgctacacttgccagcgccctagcgcccgctcctttcgctttcttcccttcctttctcgccacgttcgccggctttccccgtcaagctctaaatcgggggctccctttagggttccgatttagtgctttacggcacctcgaccccaaaaaacttgattagggtgatggttcacgtagtgggccatcgccctgatagacggtttttcgccctttgacgttggagtccacgttctttaatagtggactcttgttccaaactggaacaacactcaaccctatctcggtctattcttttgatttataagggattttgccgatttcggcctattggttaaaaaatgagctgatttaacaaaaatttaacgcgaattttaacaaaatattaacgtttacaatttcccaggtggcacttttcggggaaatgtgcgcggaacccctatttgtttatttttctaaatacattcaaatatgtatccgctcatgagacaataaccctgataaatgcttcaataatattgaaaaaggaagagtatgagtattcaacatttccgtgtcgcccttattcccttttttgcggcattttgccttcctgtttttgctcacccagaaacgctggtgaaagtaaaagatgctgaagatcagttgggtgcacgagtgggttacatcgaactggatctcaacagcggtaagatccttgagagttttcgccccgaagaacgttttccaatgatgagcacttttaaagttctgctatgtggcgcggtattatcccgtattgacgccgggcaagagcaactcggtcgccgcatacactattctcagaatgacttggttgagtactcaccagtcacagaaaagcatcttacggatggcatgacagtaagagaattatgcagtgctgccataaccatgagtgataacactgcggccaacttacttctgacaacgatcggaggaccgaaggagctaaccgcttttttgcacaacatgggggatcatgtaactcgccttgatcgttgggaaccggagctgaatgaagccataccaaacgacgagcgtgacaccacgatgcctgtagcaatggcaacaacgttgcgcaaactattaactggcgaactacttactctagcttcccggcaacaattaatagactggatggaggcggataaagttgcaggaccacttctgcgctcggcccttccggctggctggtttattgctgataaatctggagccggtgagcgtgggtctcgcggtatcattgcagcactggggccagatggtaagccctcccgtatcgtagttatctacacgacggggagtcaggcaactatggatgaacgaaatagacagatcgctgagataggtgcctcactgattaagcattggtaactgtcagaccaagtttactcatatatactttagattgatttaaaacttcatttttaatttaaaaggatctaggtgaagatcctttttgataatctcatgaccaaaatcccttaacgtgagttttcgttccactgagcgtcagaccccgtagaaaagatcaaaggatcttcttgagatcctttttttctgcgcgtaatctgctgcttgcaaacaaaaaaaccaccgctaccagcggtggtttgtttgccggatcaagagctaccaactctttttccgaaggtaactggcttcagcagagcgcagataccaaatactgtccttctagtgtagccgtagttaggccaccacttcaagaactctgtagcaccgcctacatacctcgctctgctaatcctgttaccagtggctgctgccagtggcgataagtcgtgtcttaccgggttggactcaagacgatagttaccggataaggcgcagcggtcgggctgaacggggggttcgtgcacacagcccagcttggagcgaacgacctacaccgaactgagatacctacagcgtgagctatgagaaagcgccacgcttcccgaagggagaaaggcggacaggtatccggtaagcggcagggtcggaacaggagagcgcacgagggagcttccagggggaaacgcctggtatctttatagtcctgtcgggtttcgccacctctgacttgagcgtcgatttttgtgatgctcgtcaggggggcggagcctatggaaaaacgccagcaacgcggcctttttacggttcctggccttttgctggccttttgctcacatgttctttcctgcgttatcccctgattctgtggataaccgtattaccgcctttgagtgagctgataccgctcgccgcagccgaacgaccgagcgcagcgagtcagtgagcgaggaagcggaagagcgcccaatacgcaaaccgcctctccccgcgcgttggccgattcattaatgcagctggcacgacaggtttcccgactggaaagcgggcagtgagcgcaacgcaattaatgtgagttagctcactcattaggcaccccaggctttacactttatgcttccggctcgtatgttgtgtggaattgtgagcggataacaatttcacacaggaaacagctatgaccatgattacgccaagcgcgcaattaaccctcactaaagggaacaaaagctggagctgcaagctt

SEQ ID NO: 190 - protein, 220 aa, synthetic construct
  REGION 1..220: note = Synthetic peptide
  VARIANT 143: note = Xaa can be any naturally occurring amino acid
MASAGMQILGVVLTLLGWVNGLVSCALPMWKVTAFIGNSIVVAQVVWEGLWMSCVVQSTGQMQCKVYDSLLALPQDLQAARALCVIALLVALFGLLVYLAGAKCTTCVEEKDSKARLVLTSGIVFVISGVLTLIPVCWTAHAXIRDFYNPLVAEAQKRELGASLYLGWAASGLLLLGGGLLCCTCPSGGSQGPSHYMARYSTSAPAISRGPSEYPTKNYV

SEQ ID NO: 191 - DNA, 68 bp, synthetic construct
  misc_feature 1..68: note = Synthetic polynucleotide
  source 1..68: mol_type = other DNA
cagaaactcatctcagaagaggatctggcagcaaatgatatcctggattacaaggatgacgacgataa

SEQ ID NO: 192 - DNA, 683 bp, Homo sapiens
  misc_feature 1..683: note = REGION - NCBI / NM_021195.4, 2017-06-04
  source 1..683: mol_type = genomic DNA
ccgcgatcgccatggcctctgccggaatgcagatcctgggagtcgtcctgacactgctgggctgggtgaatggcctggtctcctgtgccctgcccatgtggaaggtgaccgctttcatcggcaacagcatcgtggtggcccaggtggtgtgggagggcctgtggatgtcctgcgtggtgcagagcaccggccagatgcagtgcaaggtgtacgactcactgctggcgctgccacaggacctgcaggctgcacgtgccctctgtgtcatcgccctccttgtggccctgttcggcttgctggtctaccttgctggggccaagtgtaccacctgtgtggaggagaaggattccaaggcccgcctggtgctcacctctgggattgtctttgtcatctcaggggtcctgacgctaatccccgtgtgctggacggcgcatgccgtcatccgggacttctataaccccctggtggctgaggcccaaaagcgggagctgggggcctccctctacttgggctgggcggcctcaggccttttgttgctgggtggggggttgctgtgctgcacttgcccctcgggggggtcccagggccccagccattacatggcccgctactcaacatctgcccctgccatctctcgggggccctctgagtaccctaccaagaattacgtcacgcgtacgcgg

SEQ ID NO: 193 - DNA, 677 bp, Mus musculus
  misc_feature 1..677: note = REGION - NCBI / NM_018777.4, 2017-08-07
  source 1..677: mol_type = genomic DNA
gccgcgatcgccatggcctctactggtctgcaaatcttggggatcgtcctgaccctgcttggctgggtcaacgccctggtgtcctgtgccctgcccatgtggaaggtgaccgccttcatcggcaacagcatcgtcgtggcccagatggtgtgggaggggctgtggatgtcctgtgtggttcagagcactggccagatgcagtgcaaggtgtatgactcactgttggcgctgccccaggacctgcaggctgccagagccctctgtgttgtcaccctcctcattgtcctgcttggcctgctcgtgtacctggctggagccaagtgcactacctgtgtggaagataggaactccaagtctcgtctggtgctcatctctggcatcatctttgtcatttctggggtcctgacgctcattcctgtctgctggactgcccactctatcatccaggacttctacaaccccttggtggctgatgctcaaaagcgggagctgggggcctccctctacctgggctgggcagcctcaggccttttgctgctgggtggagggctactatgctgcgcctgctcttctggagggacccagggacccagacattacatggcctgctattctacatctgtcccacattctcggggaccctccgaatatcccaccaagaattatgtgacgcgtac

SEQ ID NO: 194 - DNA, 683 bp, synthetic construct
  misc_feature 1..683: note = Synthetic polynucleotide
  source 1..683: mol_type = other DNA
cgcgatcgccatggcctctgccggaatgcagatcctgggagtcgtcctgacactgctgggctgggtgaatggcctggtctcctgtgccctgcccatgtggaaggtgaccgctttcatcggcaacagcatcgtggtggcccaggtggtgtgggagggcctgtggatgtcctgcgtggtgcagagcaccggccagatgcagtgcaaggtgtacgactcactgctggcgctgccacaggacctgcaggctgcacgtgccctctgtgtcatcgccctccttgtggccctgttcggcttgctggtctaccttgctggggccaagtgtaccacctgtgtggaggagaaggattccaaggcccgcctggtgctcacctctgggattgtctttgtcatctcaggggtcctgacgctaatccccgtgtgctggacggcgcatgccatcatccgggacttctataaccccctggtggctgaggcccaaaagcgggagctgggggcctccctctacttgggctgggcggcctcaggccttttgttgctgggtggggggttgctgtgctgcacttgcccctcgggggggtcccagggccccagccattacatggcccgctactcaacatctgcccctgccatctctcgggggccctctgagtaccctaccaagaattacgtcacgcgtacgcggc

SEQ ID NO: 195 - DNA, 672 bp, Homo sapiens
  misc_feature 1..672: note = REGION - NCBI / NM_020982.3, 2017-04-15
  source 1..672: mol_type = genomic DNA
gccgcgatcgccatggcttcgaccggcttagaactgctgggcatgaccctggctgtgctgggctggctggggaccctggtgtcctgcgccctgcccctgtggaaggtgaccgccttcatcggcaacagcatcgtggtggcccaggtggtgtgggagggcctgtggatgtcctgcgtggtgcagagcacgggccagatgcagtgcaaggtgtacgactcactgctggctctgccgcaggacctgcaggccgcacgtgccctctgtgtcattgccctcctgctggccctgcttggcctcctggtggccatcacaggtgcccagtgtaccacgtgtgtggaggacgaaggtgccaaggcccgtatcgtgctcaccgcgggggtcatcctcctcctcgccggcatcctggtgctcatccctgtgtgctggacggcgcacgccatcatccaggacttctacaaccccctggtggctgaggccctcaagcgggagctgggggcctccctctacctgggctgggcggcggctgcactgcttatgctgggcggggggctcctctgctgcacgtgccccccgccccaggtcgagcggccccgcggacctcggctgggctactccatcccctcccgctcgggtgcatctggactggacaagagggactacgtgacgcgtacg

SEQ ID NO: 196 - DNA, 651 bp, Homo sapiens
  misc_feature 1..651: note = REGION - NCBI / NM_001305.4, 2017-07-10
  source 1..651: mol_type = genomic DNA
ccgcgatcgccatggcctccatggggctacaggtaatgggcatcgcgctggccgtcctgggctggctggccgtcatgctgtgctgcgcgctgcccatgtggcgcgtgacggccttcatcggcagcaacattgtcacctcgcagaccatctgggagggcctatggatgaactgcgtggtgcagagcaccggccagatgcagtgcaaggtgtacgactcgctgctggcactgccgcaggacctgcaggcggcccgcgccctcgtcatcatcagcatcatcgtggctgctctgggcgtgctgctgtccgtggtggggggcaagtgtaccaactgcctggaggatgaaagcgccaaggccaagaccatgatcgtggcgggcgtggtgttcctgttggccggccttatggtgatagtgccggtgtcctggacggcccacaacatcatccaagacttctacaatccgctggtggcctccgggcagaagcgggagatgggtgcctcgctctacgtcggctgggccgcctccggcctgctgctccttggcggggggctgctttgctgcaactgtccaccccgcacagacaagccttactccgccaagtattctgctgcccgctctgctgctgccagcaactacgtgacgcgtacgcggc

SEQ ID NO: 197 - DNA, 680 bp, Homo sapiens
  misc_feature 1..680: note = REGION - NCBI / NM_001306.3, 2017-07-10
  source 1..680: mol_type = genomic DNA
gccgcgatcgccatgtccatgggcctggagatcacgggcaccgcgctggccgtgctgggctggctgggcaccatcgtgtgctgcgcgttgcccatgtggcgcgtgtcggccttcatcggcagcaacatcatcacgtcgcagaacatctgggagggcctgtggatgaactgcgtggtgcagagcaccggccagatgcagtgcaaggtgtacgactcgctgctggcactgccacaggaccttcaggcggcccgcgccctcatcgtggtggccatcctgctggccgccttcgggctgctagtggcgctggtgggcgcccagtgcaccaactgcgtgcaggacgacacggccaaggccaagatcaccatcgtggcaggcgtgctgttccttctcgccgccctgctcaccctcgtgccggtgtcctggtcggccaacaccattatccgggacttctacaaccccgtggtgcccgaggcgcagaagcgcgagatgggcgcgggcctgtacgtgggctgggcggccgcggcgctgcagctgctggggggcgcgctgctctgctgctcgtgtcccccacgcgagaagaagtacacggccaccaaggtcgtctactccgcgccgcgctccaccggcccgggagccagcctgggcacaggctacgaccgcaaggactacgtcacgcgtac

SEQ ID NO: 198 - protein, 214 aa, synthetic construct
  REGION 1..214: note = Synthetic peptide
DIVLTQSPATLSVTPGNSVSLSCRASQSIGGNLHWYQQKSHESPRLLIKYASQSISGIPSRFSGSGSGTDFTLSINSVETEDFGMYFCQQSNSWPYTFGGGTKLEIKRADAAPTVSIFPPSSEQLTSGGASVVCFLNNFYPKDINVKWKIDGSERQNGVLNSWTDQDSKDSTYSMSSTLTLTKDEYERHNSYTCEATHKTSTSPIVKSFNRNEC

SEQ ID NO: 199 - protein, 444 aa, synthetic construct
  REGION 1..444: note = Synthetic peptide
DVQLQESGPSLVKPSQTLSLTCSVTGDSITSDYWSWIRKFPGNRLEYMGYVSYSGSTYYNPSLKSRISITRDTSKNQYYLDLNSVTTEDTATYYCANWDGDYWGQGTLVTVSSAAKTTAPSVYPLAPVCGDTTGSSVTLGCLVKGYFPEPVTLTWNSGSLSSGVHTFPAVLQSDLYTLSSSVTVTSSTWPSQSITCNVAHPASSTKVDKKIEPRGPTIKPCPPCKCPAPNLLGGPSVFIFPPKIKDVLMISLSPIVTCVVVDVSEDDPDVQISWFVNNVEVHTAQTQTHREDYNSTLRVVSALPIQHQDWMSGKEFKCKVNNKDLPAPIERTISKPKGSVRAPQVYVLPPPEEEMTKKQVTLTCMVTDFMPEDIYVEWTNNGKTELNYKNTEPVLDSDGSYFMYSKLRVEKKNWVERNSYSCSVVHEGLHNHHTTKSFSRTPGK

SEQ ID NO: 200 - protein, 220 aa, synthetic construct; identical to SEQ ID NO: 190
  REGION 1..220: note = Synthetic peptide
  VARIANT 143: note = Xaa can be any naturally occurring amino acid

SEQ ID NO: 201 - protein, 220 aa, synthetic construct; identical to SEQ ID NO: 190
  REGION 1..220: note = Synthetic peptide
  VARIANT 143: note = Xaa can be any naturally occurring amino acid

SEQ ID NO: 202-207 - skipped (6 entries)

SEQ ID NO: 208 - DNA, 21 bp, synthetic construct
  misc_feature 1..21: note = Synthetic polynucleotide
  source 1..21: mol_type = other DNA
tccagtgtaagttccacttac

SEQ ID NO: 209 - skipped

SEQ ID NO: 210 - DNA, 27 bp, synthetic construct
  misc_feature 1..27: note = Synthetic polynucleotide
  source 1..27: mol_type = other DNA
caccagtatcatcgttccccgctcacg

SEQ ID NO: 211 - DNA, 24 bp, synthetic construct
  misc_feature 1..24: note = Synthetic polynucleotide
  source 1..24: mol_type = other DNA
ggctacacctttactacctacacg

SEQ ID NO: 212 - DNA, 24 bp, synthetic construct
  misc_feature 1..24: note = Synthetic polynucleotide
  source 1..24: mol_type = other DNA
attaatcctagcagtggatatact

SEQ ID NO: 213 - DNA, 27 bp, synthetic construct
  misc_feature 1..27: note = Synthetic polynucleotide
  source 1..27: mol_type = other DNA
gcaaacggggattactacgtcgcttac

SEQ ID NO: 214 - DNA, 18 bp, synthetic construct
  misc_feature 1..18: note = Synthetic polynucleotide
  source 1..18: mol_type = other DNA
gagaatatttacagttat

SEQ ID NO: 215 - skipped

SEQ ID NO: 216 - DNA, 27 bp, synthetic construct
  misc_feature 1..27: note = Synthetic polynucleotide
  source 1..27: mol_type = other DNA
caacatcattatactgttccgtggacg

SEQ ID NO: 217 - DNA, 24 bp, synthetic construct
  misc_feature 1..24: note = Synthetic polynucleotide
  source 1..24: mol_type = other DNA
ggtttcactttcagtgattactgg

SEQ ID NO: 218 - DNA, 30 bp, synthetic construct
  misc_feature 1..30: note = Synthetic polynucleotide
  source 1..30: mol_type = other DNA
attagattgaaatctgataattatgcaaca

SEQ ID NO: 219 - DNA, 24 bp, synthetic construct
  misc_feature 1..24: note = Synthetic polynucleotide
  source 1..24: mol_type = other DNA
aatgatggccccccctcggggtgt

SEQ ID NO: 220 - DNA, 18 bp, synthetic construct
  misc_feature 1..18: note = Synthetic polynucleotide
  source 1..18: mol_type = other DNA
gagaatatttacagttat

SEQ ID NO: 221 - skipped

SEQ ID NO: 222 - DNA, 27 bp, synthetic construct
  misc_feature 1..27: note = Synthetic polynucleotide
  source 1..27: mol_type = other DNA
caacatcattatactgttccgtggacg

SEQ ID NO: 223 - DNA, 24 bp, synthetic construct
  misc_feature 1..24: note = Synthetic polynucleotide
  source 1..24: mol_type = other DNA
ggattcactttcagtaattactgg

SEQ ID NO: 224 - DNA, 30 bp, synthetic construct; identical to SEQ ID NO: 218
  misc_feature 1..30: note = Synthetic polynucleotide
  source 1..30: mol_type = other DNA

SEQ ID NO: 225 - DNA, 24 bp, synthetic construct
  misc_feature 1..24: note = Synthetic polynucleotide
  source 1..24: mol_type = other DNA
aatgatggccccccctcggggtgt

SEQ ID NO: 226 - DNA, 33 bp, synthetic construct
  misc_feature 1..33: note = Synthetic polynucleotide
  source 1..33: mol_type = other DNA
cagagccttgtacacagtgatggaaacacctat

SEQ ID NO: 227 - skipped

SEQ ID NO: 228 - DNA, 27 bp, synthetic construct
  misc_feature 1..27: note = Synthetic polynucleotide
  source 1..27: mol_type = other DNA
tctcaaagtacacatgttccttacacg

SEQ ID NO: 229 - DNA, 24 bp, synthetic construct
  misc_feature 1..24: note = Synthetic polynucleotide
  source 1..24: mol_type = other DNA
ggctacacctttactagctacacg

SEQ ID NO: 230 - DNA, 24 bp, synthetic construct
  misc_feature 1..24: note = Synthetic polynucleotide
  source 1..24: mol_type = other DNA
attaatcctagcagtacttatact

SEQ ID NO: 231 - DNA, 30 bp, synthetic construct
  misc_feature 1..30: note = Synthetic polynucleotide
  source 1..30: mol_type = other DNA
tcaagaggggaactgggagggtttgcttac

SEQ ID NO: 232 - DNA, 33 bp, synthetic construct
  misc_feature 1..33: note = Synthetic polynucleotide
  source 1..33: mol_type = other DNA
cagagcattgtacatagtaatggaaacacctat

SEQ ID NO: 233 - skipped

SEQ ID NO: 234 - DNA, 27 bp, synthetic construct
  misc_feature 1..27: note = Synthetic polynucleotide
  source 1..27: mol_type = other DNA
tttcaaggttcacatgttccattcacg

SEQ ID NO: 235 - DNA, 24 bp, synthetic construct
  misc_feature 1..24: note = Synthetic polynucleotide
  source 1..24: mol_type = other DNA
ggatacatattcactcactatatt

SEQ ID NO: 236 - DNA, 24 bp, synthetic construct
  misc_feature 1..24: note = Synthetic polynucleotide
  source 1..24: mol_type = other DNA
attaatccttacaatgatggtact

SEQ ID NO: 237 - DNA, 39 bp, synthetic construct
  misc_feature 1..39: note = Synthetic polynucleotide
  source 1..39: mol_type = other DNA
gcaagatactacggctacccttactattctatggactac

SEQ ID NO: 238 - DNA, 36 bp, synthetic construct
  misc_feature 1..36: note = Synthetic polynucleotide
  source 1..36: mol_type = other DNA
cagagtctgctcaacagtagaacccgaaagaactac

SEQ ID NO: 239 - skipped

SEQ ID NO: 240 - DNA, 24 bp, synthetic construct
  misc_feature 1..24: note = Synthetic polynucleotide
  source 1..24: mol_type = other DNA
aagcaatcttattatctgtacacg

SEQ ID NO: 241 - DNA, 27 bp, synthetic construct
  misc_feature 1..27: note = Synthetic polynucleotide
  source 1..27: mol_type = other DNA
ggctactccatcaccagtggttattac

SEQ ID NO: 242 - DNA, 21 bp, synthetic construct
  misc_feature 1..21: note = Synthetic polynucleotide
  source 1..21: mol_type = other DNA
atcagctacgatggtggcatt

SEQ ID NO: 243 - DNA, 30 bp, synthetic construct
  misc_feature 1..30: note = Synthetic polynucleotide
  source 1..30: mol_type = other DNA
gcaagatttggtaagggggctatggactac

SEQ ID NO: 244 - DNA, 21 bp, synthetic construct
  misc_feature 1..21: note = Synthetic polynucleotide
  source 1..21: mol_type = other DNA
tcaagtgtaagttccagttac

SEQ ID NO: 245 - skipped

SEQ ID NO: 246 - DNA, 27 bp, synthetic construct
  misc_feature 1..27: note = Synthetic polynucleotide
  source 1..27: mol_type = other DNA
caccagtatcatcgttccccacccacg

SEQ ID NO: 247 - DNA, 24 bp, synthetic construct
  misc_feature 1..24: note = Synthetic polynucleotide
  source 1..24: mol_type = other DNA
ggttactcattcactggctacacc

SEQ ID NO: 248 - DNA, 24 bp, synthetic construct
  misc_feature 1..24: note = Synthetic polynucleotide
  source 1..24: mol_type = other DNA
attaatccttacaatggtggtact

SEQ ID NO: 249 - DNA, 36 bp, synthetic construct
  misc_feature 1..36: note = Synthetic polynucleotide
  source 1..36: mol_type = other DNA
gcaagaggggtctatgattacgacggatttacttac

SEQ ID NO: 250 - DNA, 33 bp, synthetic construct; identical to SEQ ID NO: 226
  misc_feature 1..33: note = Synthetic polynucleotide
  source 1..33: mol_type = other DNA

SEQ ID NO: 251 - skipped

SEQ ID NO: 252 - DNA, 27 bp, synthetic construct
  misc_feature 1..27: note = Synthetic polynucleotide
  source 1..27: mol_type = other DNA
tctcaaagtacacatgttccttacacg

SEQ ID NO: 253 - DNA, 24 bp, synthetic construct
  misc_feature 1..24: note = Synthetic polynucleotide
  source 1..24: mol_type = other DNA
ggctacacctttactacctacacg

SEQ ID NO: 254 - DNA, 24 bp, synthetic construct
  misc_feature 1..24: note = Synthetic polynucleotide
  source 1..24: mol_type = other DNA
attaatcctcgcagtggttatagt

SEQ ID NO: 255 - DNA, 30 bp, synthetic construct; identical to SEQ ID NO: 231
  misc_feature 1..30: note = Synthetic polynucleotide
  source 1..30: mol_type = other DNA

SEQ ID NO: 256 - DNA, 18 bp, synthetic construct
  misc_feature 1..18: note = Synthetic polynucleotide
  source 1..18: mol_type = other DNA
cagaccattggtacatgg

SEQ ID NO: 257 - skipped

SEQ ID NO: 258 - DNA, 27 bp, synthetic construct
  misc_feature 1..27: note = Synthetic polynucleotide
  source 1..27: mol_type = other DNA
caacaactttacagtattcctcggacg

SEQ ID NO: 259 - DNA, 24 bp, synthetic construct
  misc_feature 1..24: note = Synthetic polynucleotide
  source 1..24: mol_type = other DNA
ggatacagattcactgactacaac

SEQ ID NO: 260 - DNA, 24 bp, synthetic construct
  misc_feature 1..24: note = Synthetic polynucleotide
  source 1..24: mol_type = other DNA
attaaccctaacaatggtggtact

SEQ ID NO: 261 - DNA, 30 bp, synthetic construct
  misc_feature 1..30: note = Synthetic polynucleotide
  source 1..30: mol_type = other DNA
gcaagagattacttgtacttctttgactgc

SEQ ID NO: 262 - DNA, 33 bp, synthetic construct
  misc_feature 1..33: note = Synthetic polynucleotide
  source 1..33: mol_type = other DNA
cagagccttgtacacagtaatggaaacacctat

SEQ ID NO: 263 - skipped

SEQ ID NO: 264 - DNA, 27 bp, synthetic construct
  misc_feature 1..27: note = Synthetic polynucleotide
  source 1..27: mol_type = other DNA
tctcaaattacacatgttccgtacacg

SEQ ID NO: 265 - DNA, 24 bp, synthetic construct
  misc_feature 1..24: note = Synthetic polynucleotide
  source 1..24: mol_type = other DNA
ggttataccttcacagactattca

SEQ ID NO: 266 - DNA, 24 bp, synthetic construct
  misc_feature 1..24: note = Synthetic polynucleotide
  source 1..24: mol_type = other DNA
ataagcactgagactggtgagcca

SEQ ID NO: 267 - DNA, 30 bp, synthetic construct
  misc_feature 1..30: note = Synthetic polynucleotide
  source 1..30: mol_type = other DNA
actagaggtctatggtcctcgtttgcttac

SEQ ID NO: 268 - DNA, 30 bp, synthetic construct
  misc_feature 1..30: note = Synthetic polynucleotide
  source 1..30: mol_type = other DNA
aaaagtgtcagtacatctggctatagttat

SEQ ID NO: 269 - skipped

SEQ ID NO: 270 - DNA, 27 bp, synthetic construct
  misc_feature 1..27: note = Synthetic polynucleotide
  source 1..27: mol_type = other DNA
cagcacagtagggagcttccgctcacg

SEQ ID NO: 271 - DNA, 24 bp, synthetic construct
  misc_feature 1..24: note = Synthetic polynucleotide
  source 1..24: mol_type = other DNA
ggattcactttcagtagctttgga

SEQ ID NO: 272 - DNA, 24 bp, synthetic construct
  misc_feature 1..24: note = Synthetic polynucleotide
  source 1..24: mol_type = other DNA
attagtagtgacagtaggaccatc

SEQ ID NO: 273 - DNA, 33 bp, synthetic construct
  misc_feature 1..33: note = Synthetic polynucleotide
  source 1..33: mol_type = other DNA
gcaagagactacggtagaacctacgaggcttac

SEQ ID NO: 274 - DNA, 18 bp, synthetic construct
  misc_feature 1..18: note = Synthetic polynucleotide
  source 1..18: mol_type = other DNA
caggacattggaggaaat

SEQ ID NO: 275 - skipped

SEQ ID NO: 276 - DNA, 27 bp, synthetic construct
  misc_feature 1..27: note = Synthetic polynucleotide
  source 1..27: mol_type = other DNA
ctacagcgtaatgcgtatccgctcact

SEQ ID NO: 277 - DNA, 24 bp, synthetic construct
  misc_feature 1..24: note = Synthetic polynucleotide
  source 1..24: mol_type = other DNA
ggattcactttcagtagttatgcc

SEQ ID NO: 278 - DNA, 21 bp, synthetic construct
  misc_feature 1..21: note = Synthetic polynucleotide
  source 1..21: mol_type = other DNA
attagaagtggtggtaccacc

SEQ ID NO: 279 - DNA, 36 bp, synthetic construct
  misc_feature 1..36: note = Synthetic polynucleotide
  source 1..36: mol_type = other DNA
gcaaaagtgggcggtaacccctatcctatggactac

SEQ ID NO: 280 - DNA, 21 bp, synthetic construct
  misc_feature 1..21: note = Synthetic polynucleotide
  source 1..21: mol_type = other DNA
tcaagtataagttccaattac

SEQ ID NO: 281 - skipped

SEQ ID NO: 282 - DNA, 27 bp, synthetic construct
  misc_feature 1..27: note = Synthetic polynucleotide
  source 1..27: mol_type = other DNA
cagcagggtagtagtataccgctcacg

SEQ ID NO: 283 - DNA, 24 bp, synthetic construct
  misc_feature 1..24: note = Synthetic polynucleotide
  source 1..24: mol_type = other DNA
ggatacgccttcagtaattacttg

SEQ ID NO: 284 - DNA, 24 bp, synthetic construct
  misc_feature 1..24: note = Synthetic polynucleotide
  source 1..24: mol_type = other DNA
attaatcctggaagtggtggtact

SEQ ID NO: 285 - DNA, 45 bp, synthetic construct
  misc_feature 1..45: note = Synthetic polynucleotide
  source 1..45: mol_type = other DNA
gcaagatcatacttcggtagaagctacccctatactatggactac

SEQ ID NO: 286 - DNA, 30 bp, synthetic construct
  misc_feature 1..30: note = Synthetic polynucleotide
  source 1..30: mol_type = other DNA
caaagtgttgattatgatggtgataattat

SEQ ID NO: 287 - skipped

SEQ ID NO: 288 - DNA, 27 bp, synthetic construct
  misc_feature 1..27: note = Synthetic polynucleotide
  source 1..27: mol_type = other DNA
cagcaaagtaatgaggatccattcacg

SEQ ID NO: 289 - DNA, 24 bp, synthetic construct
  misc_feature 1..24: note = Synthetic polynucleotide
  source 1..24: mol_type = other DNA
ggctacacattcactgattatgct

SEQ ID NO: 290 - DNA, 24 bp, synthetic construct
  misc_feature 1..24: note = Synthetic polynucleotide
  source 1..24: mol_type = other DNA
attagtacatactctggtaataca

SEQ ID NO: 291 - DNA, 39 bp, synthetic construct
  misc_feature 1..39: note = Synthetic polynucleotide
  source 1..39: mol_type = other DNA
gcaagaaggggcgattacagcctctatgctatggactac

SEQ ID NO: 292 - DNA, 36 bp, synthetic construct
  misc_feature 1..36: note = Synthetic polynucleotide
  source 1..36: mol_type = other DNA
caaagtgttttattcagttcaaatcagaaaaactac

SEQ ID NO: 293 - skipped

SEQ ID NO: 294 - DNA, 24 bp, synthetic construct
  misc_feature 1..24: note = Synthetic polynucleotide
  source 1..24: mol_type = other DNA
catcaatacctctcctcgcgcacg

SEQ ID NO: 295 - DNA, 24 bp, synthetic construct
  misc_feature 1..24: note = Synthetic polynucleotide
  source 1..24: mol_type = other DNA
ggattcactttcagtagctttgga

SEQ ID NO: 296 - DNA, 24 bp, synthetic construct
  misc_feature 1..24: note = Synthetic polynucleotide
  source 1..24: mol_type = other DNA
attagtagtgacagtaggaccatc

SEQ ID NO: 297 - DNA, 33 bp, synthetic construct; identical to SEQ ID NO: 273
  misc_feature 1..33: note = Synthetic polynucleotide
  source 1..33: mol_type = other DNA

SEQ ID NO: 298 - DNA, 30 bp, synthetic construct
  misc_feature 1..30: note = Synthetic polynucleotide
  source 1..30: mol_type = other DNA
gaaagtgttgataattatggcattagtttt

SEQ ID NO: 299 - skipped

SEQ ID NO: 300 - DNA, 27 bp, synthetic construct
  misc_feature 1..27: note = Synthetic polynucleotide
  source 1..27: mol_type = other DNA
cagcaaagtaaggaggttccgctcacg

SEQ ID NO: 301 - DNA, 24 bp, synthetic construct
  misc_feature 1..24: note = Synthetic polynucleotide
  source 1..24: mol_type = other DNA
ggattccctttcagtagctctgcc

SEQ ID NO: 302 - DNA, 21 bp, synthetic construct
  misc_feature 1..21: note = Synthetic polynucleotide
  source 1..21: mol_type = other DNA
attaatagtgatggtaacacc

SEQ ID NO: 303 - DNA, 39 bp, synthetic construct
  misc_feature 1..39: note = Synthetic polynucleotide
  source 1..39: mol_type = other DNA
acaagaaacggggactataggtacgacgagtttgcttac

SEQ ID NO: 304 - DNA, 21 bp, synthetic construct
  misc_feature 1..21: note = Synthetic polynucleotide
  source 1..21: mol_type = other DNA
tcaagtgtaagttccagttac

SEQ ID NO: 305 - skipped

SEQ ID NO: 306 - DNA, 27 bp, synthetic construct
  misc_feature 1..27: note = Synthetic polynucleotide
  source 1..27: mol_type = other DNA
caccagtatcatcgttccccacccacg

SEQ ID NO: 307 - DNA, 24 bp, synthetic construct
  misc_feature 1..24: note = Synthetic polynucleotide
  source 1..24: mol_type = other DNA
ggctacacctttactggctactgg

SEQ ID NO: 308 - DNA, 24 bp, synthetic construct
  misc_feature 1..24: note = Synthetic polynucleotide
  source 1..24: mol_type = other DNA
attaatcctagcactggttatact

SEQ ID NO: 309 - DNA, 36 bp, synthetic construct
  misc_feature 1..36: note = Synthetic polynucleotide
  source 1..36: mol_type = other DNA
gcaagagaggggattactactgtgctggttgactac

SEQ ID NO: 310 - DNA, 36 bp, synthetic construct; identical to SEQ ID NO: 292
  misc_feature 1..36: note = Synthetic polynucleotide
  source 1..36: mol_type = other DNA

SEQ ID NO: 311 - skipped

SEQ ID NO: 312 - DNA, 24 bp, synthetic construct
  misc_feature 1..24: note = Synthetic polynucleotide
  source 1..24: mol_type = other DNA
catcaatacctctcctcgcgcacg

SEQ ID NO: 313 - DNA, 24 bp, synthetic construct
  misc_feature 1..24: note = Synthetic polynucleotide
  source 1..24: mol_type = other DNA
ggttactctttcactggctacaat

SEQ ID NO: 314 - DNA, 24 bp, synthetic construct
  misc_feature 1..24: note = Synthetic polynucleotide
  source 1..24: mol_type = other DNA
attgatccttactatggtggttct

SEQ ID NO: 315 - DNA, 42 bp, synthetic construct
  misc_feature 1..42: note = Synthetic polynucleotide
  source 1..42: mol_type = other DNA
gcaagagagaggtcgggctacgttttctctgctatggactac

SEQ ID NO: 316 - DNA, 36 bp, synthetic construct; identical to SEQ ID NO: 292
  misc_feature 1..36: note = Synthetic polynucleotide
  source 1..36: mol_type = other DNA

SEQ ID NO: 317 - skipped

SEQ ID NO: 318 - DNA, 24 bp, synthetic construct
  misc_feature 1..24: note = Synthetic polynucleotide
  source 1..24: mol_type = other DNA
catcaatacctctcctcgcgcacg

SEQ ID NO: 319 - DNA, 24 bp, synthetic construct
  misc_feature 1..24: note = Synthetic polynucleotide
  source 1..24: mol_type = other DNA
ggttactcattcactggctacacc

SEQ ID NO: 320 - DNA, 24 bp, synthetic construct
  misc_feature 1..24: note = Synthetic polynucleotide
  source 1..24: mol_type = other DNA
attaatccttacaatggtgttact

SEQ ID NO: 321 - DNA, 48 bp, synthetic construct
  misc_feature 1..48: note = Synthetic polynucleotide
  source 1..48: mol_type = other DNA
acaagagatcccctttactacggctacagggactctactatggactac

SEQ ID NO: 322 - DNA, 33 bp, synthetic construct; identical to SEQ ID NO: 226
  misc_feature 1..33: note = Synthetic polynucleotide
  source 1..33: mol_type = other DNA

SEQ ID NO: 323 - skipped

SEQ ID NO: 324 - DNA, 27 bp, synthetic construct
  misc_feature 1..27: note = Synthetic polynucleotide
  source 1..27: mol_type = other DNA
tctcaaagtacacatgttccttacacg

SEQ ID NO: 325 - DNA, 24 bp, synthetic construct
  misc_feature 1..24: note = Synthetic polynucleotide
  source 1..24: mol_type = other DNA
ggctacacctttactagctacacg

SEQ ID NO: 326 - DNA, 24 bp, synthetic construct
  misc_feature 1..24: note = Synthetic polynucleotide
  source 1..24: mol_type = other DNA
attaatcctagcagtacgtatact

SEQ ID NO: 327 - DNA, 30 bp, synthetic construct; identical to SEQ ID NO: 231
  misc_feature 1..30: note = Synthetic polynucleotide
  source 1..30: mol_type = other DNA

SEQ ID NO: 328 - DNA, 18 bp, synthetic construct
  misc_feature 1..18: note = Synthetic polynucleotide
  source 1..18: mol_type = other DNA
cagggcattagaggtaat

SEQ ID NO: 329 - skipped

SEQ ID NO: 330 - DNA, 27 bp, synthetic construct
  misc_feature 1..27: note = Synthetic polynucleotide
  source 1..27: mol_type = other DNA
ctacagcgtaatgcgtatcctctcacg

SEQ ID NO: 331 - DNA, 24 bp, synthetic construct
  misc_feature 1..24: note = Synthetic polynucleotide
  source 1..24: mol_type = other DNA
ggattcactttcagtagttttgcc

SEQ ID NO: 332 - DNA, 21 bp, synthetic construct
  misc_feature 1..21: note = Synthetic polynucleotide
  source 1..21: mol_type = other DNA
attagaagtggtggtattacc

SEQ ID NO: 333 - DNA, 39 bp, synthetic construct
  misc_feature 1..39: note = Synthetic polynucleotide
  source 1..39: mol_type = other DNA
gcaagagttagtacggctacgtactatggtatggactac

SEQ ID NO: 334 - DNA, 325 bp, synthetic construct
  misc_feature 1..325: note = Synthetic polynucleotide
  source 1..325: mol_type = other DNA
caaattgttctcacccagtctccagcaatcatgtctgcatctctaggggaacgggtcaccatgacctgcactgccagctccagtgtaagttccacttactttcactggtaccaacagaagccaggatcctcccccaaactctggatttatagcacatccaacctggcttctggagtcccacgtcgcttcagtggcagtgcgtctgggacctcttactctctcacaatcagcagcatggaggctgaagatgctgccacttattattgccaccagtatcatcgttccccgctcacgttcggtgctgggaccaagctggagctgaaac

SEQ ID NO: 335 - DNA, 349 bp, synthetic construct
  misc_feature 1..349: note = Synthetic polynucleotide
  source 1..349: mol_type = other DNA
caggtccagctgcagcagtctgcagctgaactggcaagacctggggcctcagtgaagatgtcctgcaaggcttctggctacacctttactacctacacgatgcactgggtaaaacagaggcctggacagggtctggaatggattggattcattaatcctagcagtggatatactgactacaatcagaagttcaaggacaggaccacattgactgcagacaaatcctccagcacagtctacatgcaactgagtagcctgacatctgaggactctgcggtctattactgtgcaaacggggattactacgtcgcttactggggccaagggactctggtcactgtctctgcag

SEQ ID NO: 336 - DNA, 322 bp, synthetic construct
  misc_feature 1..322: note = Synthetic polynucleotide
  source 1..322: mol_type = other DNA
gacatccagatgactcagtctccagcctccctatctgcatctgtgggagaaactgtcaccatcacatgtcgaataagcgagaatatttacagttatttagcatggtatcagcagaaacagggaaaatctcctcagctcctggtctataatgcaaaaatcttagtagaaggtgtgccatcaaggttcagtggcagtggatcaggcacacagttttctctgaagatcaacagcctgcagcctgaagattttgggaattattactgtcaacatcattatactgttccgtggacgttcggtggaggcaccaaactggaaatcaaac

SEQ ID NO: 337 - DNA, 352 bp, synthetic construct
  misc_feature 1..352: note = Synthetic polynucleotide
  source 1..352: mol_type = other DNA
gaagtgaagcttgaggagtctggaggaggcttggtgcaacctggaggatccatgaaactctcctgtgttgcctctggtttcactttcagtgattactggatgaactgggtccgccagtctccagagaaggggcttgaatgggttgctcaaattagattgaaatctgataattatgcaacacattatgcggagtctgtgaaagggaggttcaccatctcaagagatgattccaaaagaagtgtctacctgcaaatgaacaacttaagggctgaagacactggaacttattactgcaatgatggccccccctcggggtgttggggccaaggcaccactctcatagtctcctcag

SEQ ID NO: 338 - DNA, 322 bp, synthetic construct
  misc_feature 1..322: note = Synthetic polynucleotide
  source 1..322: mol_type = other DNA
gacatccagatgactcagtctccagcctccctatctgcatctgtgggagaaactgtcaccatcacatgtcgaataagtgagaatatttacagttatttagcatggtatcagcagaaacagggaaaatctcctcagctcctggtctataatgcaaaaatcttagtagaaggtgtgccatcaaggttcagtggcagtggatcaggcacacagttttctctgaagatcaacagcctgcagcctgaagattttgggaattattactgtcaacatcattatactgttccgtggacgttcggtggaggcaccaaactggaaatcaaac

SEQ ID NO: 339 - DNA, 352 bp, synthetic construct
  misc_feature 1..352: note = Synthetic polynucleotide
  source 1..352: mol_type = other DNA
gaagtgaagcttgaggagtctggaggaggcttggtgcaacctggaggatccatgaaactctcctgtgttgcctctggattcactttcagtaattactggatgaactgggtccgccagtctccagagaaggggcttgaatgggttgctcaaattagattgaaatctgataattatgcaacacattatgcggagtctgtgaaagggaggttcaccatctcaagagatgattccaaaagaagtgtctacctgcaaatgaacaacttaagggctgaagacactggaacttattactgcaatgatggccccccctcggggtgttggggccaaggcaccactctcatagtctcctcag

SEQ ID NO: 340 - DNA, 337 bp, synthetic construct
  misc_feature 1..337: note = Synthetic polynucleotide
  source 1..337: mol_type = other DNA
gatgttgtgatgacccaaactccactctccctgcctgtcagtcttggagatcaagcctccatctcttgcagatctagtcagagccttgtacacagtgatggaaacacctatttaaattggtacctgcagaagccaggccagtctccaaagctcctgatctacaaagtttccaaccgtttttctggggtcccagacaggttcagtggcagtggatcagggacagatttcacactcaagatcaggagagtggaggctgaggatctgggagtttatttctgctctcaaagtacacatgttccttacacgttcggaggggggaccaagctggaaataaaac

SEQ ID NO: 341 - DNA, 352 bp, synthetic construct
  misc_feature 1..352: note = Synthetic polynucleotide
  source 1..352: mol_type = other DNA
caggtccagttgcagcagtctggggctgaactggcaagacctggggcctcagtgaagatgtcctgcaaggcttctggctacacctttactagctacacgatgcactggataaaacagagacctggacagggtcaggaatggattggatacattaatcctagcagtacttatactcattacattaagaaattcaaggacaaggccacattgactgcagacaaatcctccagcacagcctacatgcaactgcgcagcctgacatctgaggactctgcagtctattactgttcaagaggggaactgggagggtttgcttactggggccaagggactctggtcactgtctctgcag

SEQ ID NO: 342 - DNA, 337 bp, synthetic construct
  misc_feature 1..337: note = Synthetic polynucleotide
  source 1..337: mol_type = other DNA
gatgttttgatgacccaaactccactctccctgcctgtcagtcttggagatcaaccctccatctcttgcagatctagtcagagcattgtacatagtaatggaaacacctatttagattggtacctgcagaaaccaggccagtctccaaagctcctgatctacaaagtttccaaccgattttctggggtcccagacaggttcagtggcagtggatcagggacagatttcacactcaagatcagcagagtggaggctgaggatctgggagtttattactgctttcaaggttcacatgttccattcacgttcggctcggggacaaggttggaaataaaac

SEQ ID NO: 343 - DNA, 361 bp, synthetic construct
  misc_feature 1..361: note = Synthetic polynucleotide
  source 1..361: mol_type = other DNA
gaagtccagctgcagcagtctggacctgagctggtaaagcctggggcttcagtgaagatgtcctgcaaggcttctggatacatattcactcactatattatgcactgggtgaagcagaagcctgggcagggccttgagtggattggatgtattaatccttacaatgatggtactaagtacaatgagaagttcaaaggcaaggccacactgacttcagacaaatcctccagcacagcctacatggagctcagcagcctgacctctgaggactctgcggtctattactgtgcaagatactacggctacccttactattctatggactactggggtcaaggaacctcagtcaccgtctcctcag

SEQ ID NO: 344 - DNA, 337 bp, synthetic construct
  misc_feature 1..337: note = Synthetic polynucleotide
  source 1..337: mol_type = other DNA
gccattgtgatgttccagtctccatcctccctggttgtgtcagcaggagagaaggtcactatgagctgcaaatccagtcagagtctgctcaacagtagaacccgaaagaactacttggcttggtaccagcagaaaccagggcagtctcctaaactgctgatctactgggcatccactagggaatctggggtccctgatcgcttcacaggcagtggatctgggacagatttcactctcaccatcagcagtgtgcaggctgaagacctggcagtttattactgcaagcaatcttattatctgtacacgttcggaggggggaccaagctggaaataaaac

SEQ ID NO: 345 - DNA, 352 bp, synthetic construct
  misc_feature 1..352: note = Synthetic polynucleotide
  source 1..352: mol_type = other DNA
gatgtgcagcttcaggagtcaggacctggcctcgtgaaatcttctcagtctctgtctctcacctgctctgtcactggctactccatcaccagtggttattactggaaatggatccggcagtttccaggaaacaaactggaatggatgggctacatcagctacgatggtggcattaactacaacccatctctcaaaaatcgaatctccatcactcgtgacacatctaagaaccagtttttcctgaagttgaattctgtgactactgaggacacagccaaatattactgtgcaagatttggtaagggggctatggactactggggtcaaggaacctcagtcaccgtctcctcag

SEQ ID NO: 346 - DNA, 325 bp, synthetic construct
  misc_feature 1..325: note = Synthetic polynucleotide
  source 1..325: mol_type = other DNA
caaattgttctcacccagtctccagcaatcatgtctgcatctctgggggaccgggtcaccatgacctgcactgccagctcaagtgtaagttccagttacttgcactggtaccagcagaagccaggatcctcccccaaactctggatttatagcacatccaacctggcttctggagtcccagctcgcttcagtggcagtgggtctgggacctcttactctctcacaatcagcagcatggaggctgaagatgctgccacttattactgccaccagtatcatcgttccccacccacgttcggctcggggacaaagttggaaataaaac

SEQ ID NO: 347 - DNA, 358 bp, synthetic construct
  misc_feature 1..358: note = Synthetic polynucleotide
  source 1..358: mol_type = other DNA
gaggtccagctgcaacagtctggacctgagctggtgaagcctggagcttcaatgaagatatcctgcaaggcttctggttactcattcactggctacaccatgaactgggtgaagcagagccatggaaagaaccttgagtggattggacttattaatccttacaatggtggtactaactacaaccagaagttcaagggcaaggccacattaactgtagacaagtcatccagcacagcctacatggagctcctcagtctgacatctgaggactctgcagtctattactgtgcaagaggggtctatgattacgacggatttacttactggggccaagggactctggtcactgtctctgcag

SEQ ID NO: 348 - DNA, 337 bp, synthetic construct
  misc_feature 1..337: note = Synthetic polynucleotide
  source 1..337: mol_type = other DNA
gatgttgtgatgacccaaactccactctccctgcctgtcagtcttggagatcaagcctccatctcttgcagatctagtcagagccttgtacacagtgatggaaacacctatttatattggtacctgcagaagccaggccagtctccaaagctcctgatctacaaagtttccaaccgattttctggggtcccagacaggttcagtggcagtggatcagggacagatttcacactcaagatcagcagagtggaggctgaggatctgggagtttatttctgctctcaaagtacacatgttccttacacgttcggaggggggaccaagctggaaataaaac

SEQ ID NO: 349 - DNA, 352 bp, synthetic construct
  misc_feature 1..352: note = Synthetic polynucleotide
  source 1..352: mol_type = other DNA
caggtccagctgcagcagtctggggctgaactggcaagacctggggcctcagtgaagatgtcctgcaaggcttctggctacacctttactacctacacgatgcactggttaaaacagaggcctggacagggtctggaatggattggatacattaatcctcgcagtggttatagtaattacaatcagaagttcaaggacaaggccacattgactgcagacaagtcctccaacacagcctacatgcaactgaacaccctgacatctgaggactctaaagtctattactgttcaagaggggaactgggagggtttgcttactggggccaagggactctggtcactgtctctgcag

SEQ ID NO: 350 - DNA, 322 bp, synthetic construct
  misc_feature 1..322: note = Synthetic polynucleotide
  source 1..322: mol_type = other DNA
gacattcagatgacccagtctcctgcctcccagtctgcatctctgggagaaagtgtcaccatcacatgcctggcaagtcagaccattggtacatggttagcatggtatcagcagaaaccagggaaatctcctcagctcctgatttatgctgcagccagcttggcagatggggtcccatcaaggttcagtggtagtggatctggcacaagattttctttcaagatcagcagcctacaggctgaagattttgtaagttattactgtcaacaactttacagtattcctcggacgttcggtggaggcaccaagctggaaatcaaac

SEQ ID NO: 351 - DNA, 352 bp, synthetic construct
  misc_feature 1..352: note = Synthetic polynucleotide
  source 1..352: mol_type = other DNA
gaggtccagctgcaacagtctggacctgagctggtgaagcctggggcttcagtgaagatgtcctgcaaggcttctggatacagattcactgactacaacatgcactgggtgaagcagagccatggaaagagccttgagtggattggatatattaaccctaacaatggtggtactaactacaaccaaaacttcaagggcaaggccacattgactgtgaacaagtcctccagcacagcctacatggagctccgcagcctgacatcggaggattctgcagcctattactgtgcaagagattacttgtacttctttgactgctggggccaaggcaccactctcacagtctcctcag

SEQ ID NO: 352 - DNA, 337 bp, synthetic construct
  misc_feature 1..337: note = Synthetic polynucleotide
  source 1..337: mol_type = other DNA
gatgttgtgatgacccaaactccactctccctgcctgtcagtcttggagatcaagcctccatctcttgcagagctagtcagagccttgtacacagtaatggaaacacctatttacattggttcctgcagaagccaggccagtctccaaagctcctgatctacaaagtttccaaccgattttctggggtcccagacaggttcagtggcagtggatcacggacagatttcacactcaagatcagcagagtggaggctgaggatctgggagtttatttctgctctcaaattacacatgttccgtacacgttcggaggggggaccaagctggaaataaaac

SEQ ID NO: 353 - DNA, 352 bp, synthetic construct
  misc_feature 1..352: note = Synthetic polynucleotide
  source 1..352: mol_type = other DNA
caaatccagttggtgcagtctggacctgcgctgaagaagcctggagagacagtcaagatctcctgcaaggcttctggttataccttcacagactattcaatgcactggataaagcaggctccaggaaagggtttaaagtggatgggctggataagcactgagactggtgagccaacatatgcagatggcttcaagggacggtttgacttctctttggaaacctctgccgacactgcctatttgtccatcaacaacctcacaaatgaggacacggctacatatttctgtactagaggtctatggtcctcgtttgcttactggggccaagggactctggtcactgtctctgcag

SEQ ID NO: 354 - DNA, 334 bp, synthetic construct
  misc_feature 1..334: note = Synthetic polynucleotide
  source 1..334: mol_type = other DNA
gacattgtgctgacacagtctcctgcttccttagctgtatctctggggcagagggccaccatctcatgcagggccagcaaaagtgtcagtacatctggctatagttatatacactggtaccaacagaaaccaggacagccacccaaactcctcatctatcttgcatccaacctagaatctggggtccctgccaggttcagtggcagtgggtctgggacagacttcaccctcaacatccatcctgtggaggaggaggatgctgcaacctattactgtcagcacagtagggagcttccgctcacgttcggtgctgggaccaagctggagctgaaac

SEQ ID NO: 355 - DNA, 355 bp, synthetic construct
  misc_feature 1..355: note = Synthetic polynucleotide
  source 1..355: mol_type = other DNA
gatgtgcagctggtggagtctgggggaggcttggtgcagcctagagggtcccggaaactctcctgtgcagcctctggattcactttcagtagctttggaatgcactgggttcgtcaggctccagagaaggggctggagtgggtcgcatacattagtagtgacagtaggaccatctattatgcagacacagtgaagggccgattcaccatctccagagacaatcccacgaacaccctgttcctgcaaatgaccagtctcaggtctgaggacacggccatgtattactgtgcaagagactacggtagaacctacgaggcttactggggccaagggactctggtcactgtctctgcag

SEQ ID NO: 356 - DNA, 322 bp, synthetic construct
  misc_feature 1..322: note = Synthetic polynucleotide
  source 1..322: mol_type = other DNA
gacatccagatgattcagtctccatcgtccatgtttgcctctctgggagacagagtcagtctctcttgtcgggctagtcaggacattggaggaaatttagactggtatcagcagaaaccaggtggaactattaaactcctgatctactccacatccaatttaaattctggtgtcccatcaaggttcagtggcagtgggtctgggtcagattattctctcaccatcaccagcctggagtctgaagattttgcagactattactgtctacagcgtaatgcgtatccgctcactttcggtgctgggaccaagctggagctgaaac

SEQ ID NO: 357 - DNA, 355 bp, synthetic construct
  misc_feature 1..355: note = Synthetic polynucleotide
  source 1..355: mol_type = other DNA
gaagtgaaactgatggagtctgggggagacttagtgaagcctggagggtccctgaaactctcctgtgcagcctctggattcactttcagtagttatgccatgtcttgggttcgccagactccagagaagaggctggagtgggtcgcgtccattagaagtggtggtaccacctactatccagacagtgtgaagggccgattcaccatctccagagataatgccaggaacatcctgtacctgcgaatgagtagtctgaggtctgaggacacggccatatattactgtgcaaaagtgggcggtaacccctatcctatggactactggggtcaaggaacctcagtcaccgtctcctcag

SEQ ID NO: 358 - DNA, 325 bp, synthetic construct
  misc_feature 1..325: note = Synthetic polynucleotide
  source 1..325: mol_type = other DNA
gaaattgtgctcacccagtctccaaccaccatggctgcatctcccggggagaagatcactatcacctgcagtgccagctcaagtataagttccaattacttgcattggtatcagcagaagccaggattctcccctaaactcttgatttataggacatccaatctggcttctggagtcccagctcgcttcagtggcagtgggtctgggacctcttactctctcacaattggcaccatggaggctgaagatgttgccacttactactgccagcagggtagtagtataccgctcacgttcggtgctgggaccaagctggagctgaaac

SEQ ID NO: 359 - DNA, 367 bp, synthetic construct
  misc_feature 1..367: note = Synthetic polynucleotide
  source 1..367: mol_type = other DNA
caggtccagctgcagcagtctggagctgagctggtaaggcctgggacttcagtgaaggtgtcctgcaaggcttctggatacgccttcagtaattacttgatagagtgggttaagcagaggcctggacagggccttgagtggattggagtgattaatcctggaagtggtggtactaactacaatgagaagttcaagggcaaggcaacaatgactgcagacaaatcctccagcactgcctacatgcacctcagcaacctgacatctgaggactctgtggtctatttctgtgcaagatcatacttcggtagaagctacccctatactatggactactggggtcaaggaacctcagtcaccgtctcctcag

SEQ ID NO: 360 - DNA, 334 bp, synthetic construct
  misc_feature 1..334: note = Synthetic polynucleotide
  source 1..334: mol_type = other DNA
gatattgtgctgacccaatctccagcttctttggctgtgtctctagggcagagggccaccatctcctgcaaggccagccaaagtgttgattatgatggtgataattatgtgaactggtaccaacagaaagtaggacagccacccaaactcctcatctctgctgcatccaatctagaatctgggatcccagccaggtttagtggcagtgggtctgggacagacttcaccctcaacatccatcctgtggaggaggaggatgctgcaacctattactgtcagcaaagtaatgaggatccattcacgttcggctcggggacaaagttggaaataaaac

SEQ ID NO: 361 - DNA, 361 bp, synthetic construct
  misc_feature 1..361: note = Synthetic polynucleotide
  source 1..361: mol_type = other DNA
caggtccagctgcagcagtctgggcctgagctggtgaggcctggggtctcagtgaagatttcctgcaagggttccggctacacattcactgattatgctatgcactgggtgaagcagagtcatgcaaagagtctagagtggattggagttattagtacatactctggtaatacaaactacaaccagaagtttcaggacaaggccaccatgactgtagacaaatcctccagcacagcctatatggcacttgccagattgacatctgacgattctgccatctattactgtgcaagaaggggcgattacagcctctatgctatggactactggggtcaaggaacctcagtcaccgtctcctcag

SEQ ID NO: 362 - DNA, 337 bp, synthetic construct
  misc_feature 1..337: note = Synthetic polynucleotide
  source 1..337: mol_type = other DNA
aacattatgatgacacagtcgccatcatctctggctgtgtctgcaggagaaaaggtcactatgagctgtaagtccagtcaaagtgttttattcagttcaaatcagaaaaactacttggcctggtaccagcagaaaccagggcagtctcctagactgctgatctactgggcatccactagggaatctggtgtccctgatcgcttcacaggcagtggatctgggacagattttactcttaccatcagcaatgttcaagctgaagacctggcagtttattactgtcatcaatacctctcctcgcgcacgttcggtgctgggaccaagctggagctgaaac

SEQ ID NO: 363 - DNA, 355 bp, synthetic construct; identical to SEQ ID NO: 355
  misc_feature 1..355: note = Synthetic polynucleotide
  source 1..355: mol_type = other DNA

SEQ ID NO: 364 - DNA, 334 bp, synthetic construct
  misc_feature 1..334: note = Synthetic polynucleotide
  source 1..334: mol_type = other DNA
gacattgtgctgacccaatctccagcttctttggctctgtctctagggcagagggccaccatctcctgcagagccagcgaaagtgttgataattatggcattagttttatgaactggttccaacagaaacccggacagccacccaaactcctcatctatgctgcatccaaccaaggatccggggtccctgccaggtttagtggcagtgggtctgggacagacttcagcctcaacatccatcctatggaggaggatgatactgcaatgtatttctgtcagcaaagtaaggaggttccgctcacgttcggtgctgggaccaagctggagctgaaac

SEQ ID NO: 365 - DNA, 358 bp, synthetic construct
  misc_feature 1..358: note = Synthetic polynucleotide
  source 1..358: mol_type = other DNA
gaagtgaggctggtggagtctgggggaggcttgatgcagcctggagggtccctgaaactcccctgtgcagcctctggattccctttcagtagctctgccatgtcttgggttcgccagactccagagaagaggctggagtgggtcgcatccattaatagtgatggtaacacctactatcccgacagtgtgaagggccgattcaccatctccagagatagtgccaggaacatcctgtacctccaaatgagcagtctgaggtctgaggacacggccatgtattactgtacaagaaacggggactataggtacgacgagtttgcttactggggccaagggactctggtcactgtctctgcag

SEQ ID NO: 366 - DNA, 325 bp, synthetic construct
  misc_feature 1..325: note = Synthetic polynucleotide
  source 1..325: mol_type = other DNA
caaattgttctcacccagtctccagcaatcatgtctgcatctctaggggaacgggtcaccatgacctgcactgccagctcaagtgtaagttccagttacttgcactggtaccagcagaagccaggatcctcccccaaactctggatttatagcacatccaacctggcttctggagtcccagctcgcttcagtggcagtgggtctgggacctcttactctctcacaatcagcagcatggaggctgaagatgctgccacttattactgccaccagtatcatcgttccccacccacgttcggagctgggaccaagctggagctgaaac

SEQ ID NO: 367 - DNA, 358 bp, synthetic construct
  misc_feature 1..358: note = Synthetic polynucleotide
  source 1..358: mol_type = other DNA
caggtccagcttcagcagtctggggctgaactggcaaaacctggggcctcagtgaagatgtcctgcaaggcttctggctacacctttactggctactggatgcactgggtaaaacagaggcctggacagggtctggaatggcttggatacattaatcctagcactggttatactgagtccaatcagaagttcaaggacaaggccacattgactgcagacaaatcctccaccacagcctacatgcaactgagaagcctgacacctgaggactctgcagtctattactgtgcaagagaggggattactactgtgctggttgactactggggccaaggcaccactctcacagtctcctcag

SEQ ID NO: 368 - DNA, 337 bp, synthetic construct; identical to SEQ ID NO: 362
  misc_feature 1..337: note = Synthetic polynucleotide
  source 1..337: mol_type = other DNA

SEQ ID NO: 369 - DNA, 364 bp, synthetic construct
  misc_feature 1..364: note = Synthetic polynucleotide
  source 1..364: mol_type = other DNA
caggtgcagctgaagcagtctggacctgagctggagaagcctggcgcttcagtgaagatatcctgcaaggcttctggttactctttcactggctacaatatgaactgggtgaagcagagcaatggaaagagccttgagtggattggaaatattgatccttactatggtggttctacctacaaccagaagttcacgggcaaggccacattgactgtagacaaatcctccagcacagcctacatgcagctcaagagcctgacatctgaggactctgcagtgtattactgtgcaagagagaggtcgggctacgttttctctgctatggactactggggtcaaggaacctcagtcaccgtctcctcag

SEQ ID NO: 370 - DNA, 337 bp, synthetic construct; identical to SEQ ID NO: 362
  misc_feature 1..337: note = Synthetic polynucleotide
  source 1..337: mol_type = other DNA

SEQ ID NO: 371 - DNA, 370 bp, synthetic construct
  misc_feature 1..370: note = Synthetic polynucleotide
  source 1..370: mol_type = other DNA
gaggtccagctgcaacagtctggacctgagctggtgaagcctggaggttcaatgaagatatcctgcaaggcttctggttactcattcactggctacaccatgaactgggtgaagcggagccatggaaagaaccttgagtggattggacttattaatccttacaatggtgttactacctacaaccagaacttcaagggcaaggccacattagctgtagacaagtcatccagcacagcctacatggagctcctcggtctgacatctgaggactctgcagtctattactgtacaagagatcccctttactacggctacagggactctactatggactactggggtcaaggaacctcagtcaccgtctcctcag

SEQ ID NO: 372 - DNA, 337 bp, synthetic construct; identical to SEQ ID NO: 340
  misc_feature 1..337: note = Synthetic polynucleotide
  source 1..337: mol_type = other DNA

SEQ ID NO: 373 - DNA, 352 bp, synthetic construct
  misc_feature 1..352: note = Synthetic polynucleotide
  source 1..352: mol_type = other DNA
gaggtccagctgcagcagtctggggctgaactggcaagacctggggcctcagtgaagatgtcctgcaaggcttctggctacacctttactagctacacgatgcactggataaaacagagacctggacagggtcaggaatggattggatacattaatcctagcagtacgtatactcattacattaagaagttcaaggacaaggccacattgactgcagacaaatcctccagcacagcctacatgcaactgcgcagcctgacatctgaggactctgcagtctattactgttcaagaggggaactgggagggtttgcttactggggccaagggactctggtcactgtctctgcag

SEQ ID NO: 374 - DNA, 322 bp, synthetic construct
  misc_feature 1..322: note = Synthetic polynucleotide
  source 1..322: mol_type = other DNA
gacatccagatgattcagtctccatcgtccatgtttgcctctctgggagacagagtcagtctctcttgtcgggctagtcagggcattagaggtaatttagactggtatcagcagaaaccaggtggaactattaaactcctgatctactccacatccattttaaattctggtgtcccatcaaggttcagtggcagtgggtctgggtcagattattctctcaccatcaccagcctagagtctgaagattttgcagactattactgtctacagcgtaatgcgtatcctctcacgttcggttctgggaccaagctggagctgaaac

SEQ ID NO: 375 - DNA, 358 bp, synthetic construct
  misc_feature 1..358: note = Synthetic polynucleotide
  source 1..358: mol_type = other DNA
gaagtgaagttggtggagtctgggggaggcttaatgaagcctggagggtccctgaaactctcctgtgcggcctctggattcactttcagtagttttgccttgtcttgggttcgccagactccagagaagaggctggagtgggtcgcatccattagaagtggtggtattacctaccatgcagacagtgtgaagggccgattcaccatctccagagataatgccgggaacatcctgtacctgcaaatgaacagtctgaggtctgaggacacggccatgtatttctgtgcaagagttagtacggctacgtactatggtatggactactggggtcaaggaacctcagtcaccgtctcctcag

SEQ ID NO: 376 - protein, 116 aa, synthetic construct
  REGION 1..116: note = Synthetic peptide
QVQLVQSGAEVKKPGASVKVSCKASGYTFTTYTMHWVRQAPGQGLEWMGFINPSSGYTDYAQKFQGRVTMTRDTSTSTVYMELSSLRSEDTAVYYCARGDYYVAYWGQGTLVTVSS

SEQ ID NO: 377 - protein, 116 aa, synthetic construct
  REGION 1..116: note = Synthetic peptide
QVQLVQSGAEVKKPGASVKVSCKASGYTFTTYTMHWVRQAPGQGLEWMGFINPSSGYTDYAQKFQGRVTMTADTSTSTVYMELSSLRSEDTAVYYCANGDYYVAYWGQGTLVTVSS

SEQ ID NO: 378 - protein, 116 aa, synthetic construct
  REGION 1..116: note = Synthetic peptide
QVQLVQSGAEVKKPGASVKMSCKASGYTFTTYTMHWVRQAPGQGLEWIGFINPSSGYTDYAQKFQGRVTLTADTSTSTVYMELSSLRSEDTAVYYCANGDYYVAYWGQGTLVTVSS

SEQ ID NO: 379 - protein, 116 aa, synthetic construct
  REGION 1..116: note = Synthetic peptide
QVQLVQSGAEVKKPGASVKMSCKASGYTFTTYTMHWVRQAPGQGLEWIGFINPSSGYTDYAQKFQGRVTLTADKSTSTVYMELSSLRSEDTAVYYCANGDYYVAYWGQGTLVTVSS

SEQ ID NO: 380 - protein, 108 aa, synthetic construct
  REGION 1..108: note = Synthetic peptide
DIQMTQSPSSLSASVGDRVTITCTASSSVSSTYFHWYQQKPGKAPKLLIYSTSNLASGVPSRFSGSGSGTDFTLTISSLQPEDFATYYCHQYHRSPLTFGQGTKLEIK

SEQ ID NO: 381 - protein, 108 aa, synthetic construct
  REGION 1..108: note = Synthetic peptide
DIQMTQSPSSLSASVGDRVTITCTASSSVSSTYFHWYQQKPGKAPKLLIYSTSNLASGVPSRFSGSGSGTDYTLTISSLQPEDFATYYCHQYHRSPLTFGQGTKLEIK

SEQ ID NO: 382 - protein, 108 aa, synthetic construct
  REGION 1..108: note = Synthetic peptide
DIQLTQSPSSLSASVGDRVTMTCTASSSVSSTYFHWYQQKPGKAPKLLIYSTSNLASGVPSRFSGSGSGTDYTLTISSMQPEDAATYYCHQYHRSPLTFGQGTKLEIK

SEQ ID NO: 383 - protein, 108 aa, synthetic construct
  REGION 1..108: note = Synthetic peptide
DIQLTQSPSSLSASVGDRVTMTCTASSSVSSTYFHWYQQKPGKAPKLWIYSTSNLASGVPSRFSGSGSGTDYTLTISSMQPEDAATYYCHQYHRSPLTFGQGTKLEIK

SEQ ID NO: 384 - protein, 117 aa, synthetic construct
  REGION 1..117: note = Synthetic peptide
EVQLLESGGGLVQPGGSLRLSCAASGFTFSNYWMNWVRQAPGKGLEWVSQIRLKSDNYATHYADSVKGRFTISRDNSKNTLYLQMNSLRAEDTAVYYCAKGPPSGCWGQGTLVTVSS

SEQ ID NO: 385 - protein, 117 aa, synthetic construct
  REGION 1..117: note = Synthetic peptide
EVQLLESGGGLVQPGGSMRLSCAASGFTFSNYWMNWVRQAPGKGLEWVAQIRLKSDNYATHYADSVKGRFTISRDDSKNTVYLQMNSLRAEDTGVYYCNDGPPSGCWGQGTLLTVSS

SEQ ID NO: 386 - protein, 117 aa, synthetic construct
  REGION 1..117: note = Synthetic peptide
EVQLLESGGGLVQPGGSMRLSCAASGFTFSNYWMNWVRQAPGKGLEWVAQIRLKSDNYATHYADSVKGRFTISRDDSKNTVYLQMNSLRAEDTGVYYCNDGPPSGYWGQGTLLTVSS

SEQ ID NO: 387 - protein, 117 aa, synthetic construct
  REGION 1..117: note = Synthetic peptide
EVQLLESGGGLVQPGGSMRLSCAASGFTFSNYWMNWVRQAPGKGLEWVAQIRLKSDNYATHYADSVKGRFTISRDDSKNTVYLQMNSLRAEDTGVYYCNDGPPSGSWGQGTLLTVSS

SEQ ID NO: 388 - protein, 107 aa, synthetic construct
  REGION 1..107: note = Synthetic peptide
DIQMTQSPSSLSASVGDRVTITCRISENIYSYLAWYQQKPGKAPKLLIYNAKILVEGVPSRFSGSGSGTDFTLTISSLQPEDFATYYCQHHYTVPWTFGQGTKLEIK

SEQ ID NO: 389 - protein, 107 aa, synthetic construct
  REGION 1..107: note = Synthetic peptide
DIQMTQSPSSLSASVGDRVTITCRISENIYSYLAWYQQKPGKAPKLLVYNAKILVEGVPSRFSGSGSGTDFTLTISSLQPEDFGTYYCQHHYTVPWTFGQGTKLEIK

SEQ ID NO: 390 - protein, 107 aa, synthetic construct
  REGION 1..107: note = Synthetic peptide
DIQMTQSPSSLSASVGDRVTITCRISENIYSYLAWYQQKPGKAPKLLVYNAKSLVEGVPSRFSGSGSGTDFTLTISSLQPEDFGTYYCQHHYTVPWTFGQGTKLEIK

SEQ ID NO: 391 - protein, 117 aa, synthetic construct
  REGION 1..117: note = Synthetic peptide
QVQLVQSGAEVKKPGASVKVSCKASGYTFTSYTMHWVRQAPGQGLEWMGYINPSSTYTHYAQKFQGRVTMTRDTSTSTVYMELSSLRSEDTAVYYCARGELGGFAYWGQGTLVTVSS

SEQ ID NO: 392 - protein, 117 aa, synthetic construct
  REGION 1..117: note = Synthetic peptide
QVQLVQSGAEVKKPGASVKVSCKASGYTFTSYTMHWVRQAPGQGLEWMGYINPSSTYTHYAQKFQGRVTMTADTSTSTVYMELSSLRSEDTAVYYCSRGELGGFAYWGQGTLVTVSS

SEQ ID NO: 393 - protein, 117 aa, synthetic construct
  REGION 1..117: note = Synthetic peptide
QVQLVQSGAEVKKPGASVKMSCKASGYTFTSYTMHWIRQAPGQGLEWIGYINPSSTYTHYAQKFQGRATLTADTSTSTAYMELSSLRSEDTAVYYCSRGELGGFAYWGQGTLVTVSS

SEQ ID NO: 394 - protein, 117 aa, synthetic construct
  REGION 1..117: note = Synthetic peptide
QVQLVQSGAEVKKPGASVKMSCKASGYTFTSYTMHWIRQAPGQGQEWIGYINPSSTYTHYAQKFQGRATLTADTSTSTAYMELSSLRSEDTAVYYCSRGELGGFAYWGQGTLVTVSS

SEQ ID NO: 395 - protein, 117 aa, synthetic construct
  REGION 1..117: note = Synthetic peptide
QVQLVQSGAEVKKPGASVKMSCKASGYTFTSYTMHWIRQAPGQGLEWIGYINPSSTYTHYAQKFQGRATLTADKSTSTAYMELSSLRSEDTAVYYCSRGELGGFAYWGQGTLVTVSS

SEQ ID NO: 396 - protein, 117 aa, synthetic construct
  REGION 1..117: note = Synthetic peptide
QVQLVQSGAEVKKPGASVKMSCKASGYTFTSYTMHWIRQAPGQGQEWIGYINPSSTYTHYAQKFQGRATLTADKSTSTAYMELSSLRSEDTAVYYCSRGELGGFAYWGQGTLVTVSS

SEQ ID NO: 397 - protein, 112 aa, synthetic construct
  REGION 1..112: note = Synthetic peptide
DVVMTQSPLSLPVTLGQPASISCRSSQSLVHSDGNTYLNWFQQRPGQSPRRLIYKVSNRFSGVPDRFSGSGSGTDFTLKISRVEAEDVGVYYCSQSTHVPYTFGQGTKLEIK

SEQ ID NO: 398 - protein, 112 aa, synthetic construct
  REGION 1..112: note = Synthetic peptide
DVVMTQSPLSLPVTLGQPASISCRSSQSLVHSDGNTYLNWYQQRPGQSPRLLIYKVSNRFSGVPDRFSGSGSGTDFTLKISRVEAEDVGVYYCSQSTHVPYTFGQGTKLEIK

SEQ ID NO: 399 - protein, 112 aa, synthetic construct
  REGION 1..112: note = Synthetic peptide
DVVMTQSPLSLPVTLGQPASISCRSSQSLVHSEGNTYLNWYQQRPGQSPRLLIYKVSNRFSGVPDRFSGSGSGTDFTLKISRVEAEDVGVYYCSQSTHVPYTFGQGTKLEIK

SEQ ID NO: 400 - protein, 112 aa, synthetic construct
  REGION 1..112: note = Synthetic peptide
DVVMTQSPLSLPVTLGQPASISCRSSQSLVHSSGNTYLNWYQQRPGQSPRLLIYKVSNRFSGVPDRFSGSGSGTDFTLKISRVEAEDVGVYYCSQSTHVPYTFGQGTKLEIK

SEQ ID NO: 401 - protein, 112 aa, synthetic construct
  REGION 1..112: note = Synthetic peptide
DVVMTQSPLSLPVTLGQPASISCRSSQSLVHSEGSTYLNWYQQRPGQSPRLLIYKVSNRFSGVPDRFSGSGSGTDFTLKISRVEAEDVGVYYCSQSTHVPYTFGQGTKLEIK

SEQ ID NO: 402 - protein, 112 aa, synthetic construct
  REGION 1..112: note = Synthetic peptide
DVVMTQSPLSLPVTLGQPASISCRSSQSLVHSSGSTYLNWYQQRPGQSPRLLIYKVSNRFSGVPDRFSGSGSGTDFTLKISRVEAEDVGVYYCSQSTHVPYTFGQGTKLEIK

SEQ ID NO: 403 - protein, 117 aa, synthetic construct
  REGION 1..117: note = Synthetic peptide
QVQLVQSGAEVKKPGASVKVSCKASGYRFTDYNMHWVRQAPGQGLEWMGYINPNNGGTNYAQKFQGRVTMTRDTSTSTVYMELSSLRSEDTAVYYCARDYLYFFDCWGQGTLVTVSS

SEQ ID NO: 404 - protein, 117 aa, synthetic construct
  REGION 1..117: note = Synthetic peptide
QVQLVQSGAEVKKPGASVKVSCKASGYRFTDYNMHWVRQAPGQGLEWMGYINPNNGGTNYAQKFQGRVTMTVDTSTSTVYMELSSLRSEDTAVYYCARDYLYFFDCWGQGTLVTVSS

SEQ ID NO: 405 - protein, 117 aa, synthetic construct
  REGION 1..117: note = Synthetic peptide
QVQLVQSGAEVKKPGASVKMSCKASGYRFTDYNMHWVRQAPGQGLEWIGYINPNNGGTNYAQKFQGRATLTVDTSTSTAYMELSSLRSEDTAVYYCARDYLYFFDCWGQGTLLTVSS

SEQ ID NO: 406 - protein, 117 aa, synthetic construct
  REGION 1..117: note = Synthetic peptide
QVQLVQSGAEVKKPGASVKMSCKASGYRFTDYNMHWVRQAPGQGLEWIGYINPNNGGTNYAQKFQGRATLTVDKSTSTAYMELSSLRSEDTAVYYCARDYLYFFDCWGQGTLLTVSS

SEQ ID NO: 407 - protein, 117 aa, synthetic construct
  REGION 1..117: note = Synthetic peptide
QVQLVQSGAEVKKPGASVKMSCKASGYRFTDYNMHWVRQAPGQGLEWIGYINPNNGGTNYAQKFQGRATLTVNKSTSTAYMELSSLRSEDTAVYYCARDYLYFFDCWGQGTLLTVSS

SEQ ID NO: 408 - protein, 117 aa, synthetic construct
  REGION 1..117: note = Synthetic peptide
QVQLVQSGAEVKKPGASVKMSCKASGYRFTDYNMHWVRQAPGQGLEWIGYINPNNGGTNYAQKFQGRATLTVNTSTSTAYMELSSLRSEDTAVYYCARDYLYFFDCWGQGTLLTVSS

SEQ ID NO: 409 - protein, 107 aa, synthetic construct
  REGION 1..107: note = Synthetic peptide
DIQMTQSPSSLSASVGDRVTITCLASQTIGTWLAWYQQKPGKAPKLLIYAAASLADGVPSRFSGSGSGTDFTLTISSLQPEDFATYYCQQLYSIPRTFGQGTKLEIK

SEQ ID NO: 410 - protein, 107 aa, synthetic construct
  REGION 1..107: note = Synthetic peptide
DIQMTQSPSSLSASVGDRVTITCLASQTIGTWLAWYQQKPGKAPKLLIYAAASLADGVPSRFSGSGSGTDFTFTISSLQPEDFVTYYCQQLYSIPRTFGQGTKLEIK

SEQ ID NO: 411 - protein, 107 aa, synthetic construct
  REGION 1..107: note = Synthetic peptide
DIQMTQSPSSLSASVGDRVTITCRASQTIGTWLAWYQQKPGKAPKLLIYAAASLADGVPSRFSGSGSGTDFTFTISSLQPEDFVTYYCQQLYSIPRTFGQGTKLEIK

SEQ ID NO: 412 - protein, 118 aa, synthetic construct
  REGION 1..118: note = Synthetic peptide
EVQLVESGGGLVQPGGSLRLSCAASGFTFSSFGMHWVRQAPGKGLEWVSYISSDSRTIYYADSVKGRFTISRDNAKNSLYLQMNSLRAEDTAVYYCARDYGRTYEAYWGQGTLVTVSS

SEQ ID NO: 413 - protein, 118 aa, synthetic construct
  REGION 1..118: note = Synthetic peptide
EVQLVESGGGLVQPGGSLRLSCAASGFTFSSFGMHWVRQAPGKGLEWVAYISSDSRTIYYADSVKGRFTISRDNAKNSLYLQMNSLRAEDTAVYYCARDYGRTYEAYWGQGTLVTVSS

SEQ ID NO: 414 - protein, 111 aa, synthetic construct
  REGION 1..111: note = Synthetic peptide
DIVMTQSPDSLAVSLGERATINCRASKSVSTSGYSYIHWYQQKPGQPPKLLIYLASNLESGVPDRFSGSGSGTDFTLTISSLQAEDVAVYYCQHSRELPLTFGQGTKLEIK

SEQ ID NO: 415 - protein, 111 aa, synthetic construct
  REGION 1..111: note = Synthetic peptide
DIVLTQSPDSLAVSLGERATINCRASKSVSTSGYSYIHWYQQKPGQPPKLLIYLASNLESGVPDRFSGSGSGTDFTLTISSVQAEDVAVYYCQHSRELPLTFGQGTKLELK

SEQ ID NO: 416 - protein, 121 aa, synthetic construct
  REGION 1..121: note = Synthetic peptide
QVQLVQSGAEVKKPGASVKVSCKASGYSFTGYNMNWVRQAPGQGLEWMGNIDPYYGGSTYAQKFQGRVTMTRDTSTSTVYMELSSLRSEDTAVYYCARERSGYVFSAMDYWGQGTLVTVSS

SEQ ID NO: 417 - protein, 121 aa, synthetic construct
  REGION 1..121: note = Synthetic peptide
QVQLVQSGAEVKKPGASVKVSCKASGYSFTGYNMNWVRQAPGQGLEWMGNIDPYYGGSTYAQKFQGRVTMTVDTSTSTVYMELSSLRSEDTAVYYCARERSGYVFSAMDYWGQGTLVTVSS

SEQ ID NO: 418 - protein, 121 aa, synthetic construct
  REGION 1..121: note = Synthetic peptide
QVQLVQSGAEVKKPGASVKISCKASGYSFTGYNMNWVRQAPGQGLEWIGNIDPYYGGSTYAQKFQGRATLTVDTSTSTAYMELSSLRSEDTAVYYCARERSGYVFSAMDYWGQGTLVTVSS

SEQ ID NO: 419 - protein, 121 aa, synthetic construct
  REGION 1..121: note = Synthetic peptide
QVQLVQSGAEVKKPGASVKISCKASGYSFTGYNMNWVRQAPGQGLEWIGNIDPYYGGSTYAQKFQGRATLTVDKSTSTAYMELSSLRSEDTAVYYCARERSGYVFSAMDYWGQGTLVTVSS

SEQ ID NO: 420 - protein, 112 aa, synthetic construct
  REGION 1..112: note = Synthetic peptide
DIVMTQSPDSLAVSLGERATINCKSSQSVLFSSNQKNYLAWYQQKPGQPPKLLIYWASTRESGVPDRFSGSGSGTDFTLTISSLQAEDVAVYYCHQYLSSRTFGQGTKLEIK

SEQ ID NO: 421 - protein, 112 aa, synthetic construct
  REGION 1..112: note = Synthetic peptide
DIVMTQSPDSLAVSLGERVTMNCKSSQSVLFSSNQKNYLAWYQQKPGQPPKLLIYWASTRESGVPDRFSGSGSGTDFTLTISSVQAEDVAVYYCHQYLSSRTFGQGTKLEIK

SEQ ID NO: 422 - protein, 117 aa, synthetic construct
  REGION 1..117: note = Synthetic peptide
EVQLLESGGGLVQPGGSMRLSCAASGFTFSNYWMNWVRQAPGKGLEWVAQIRLKSDNYATHYADSVKGRFTISRDDSKNTVYLQMNSLRAEDTGVYYCNDGPPSGAWGQGTLLTVSS

SEQ ID NO: 423 - protein, 117 aa, synthetic construct
  REGION 1..117: note = Synthetic peptide
QVQLVQSGAEVKKPGASVKVSCKASGYTFTSYTMHWVRQAPGQGLEWMGYINPSSTYTHYIKKFKDRVTMTADTSTSTVYMELSSLRSEDTAVYYCSRGELGGFAYWGQGTLVTVSS

SEQ ID NO: 424 - protein, 117 aa, synthetic construct
  REGION 1..117: note = Synthetic peptide
QVQLVQSGAEVKKPGASVKMSCKASGYTFTSYTMHWIRQAPGQGLEWIGYINPSSTYTHYIKKFKDRATLTADTSTSTAYMELSSLRSEDTAVYYCSRGELGGFAYWGQGTLVTVSS

SEQ ID NO: 425 - protein, 117 aa, synthetic construct
  REGION 1..117: note = Synthetic peptide
QVQLVQSGAEVKKPGASVKMSCKASGYTFTSYTMHWIRQAPGQGQEWIGYINPSSTYTHYIKKFKDRATLTADTSTSTAYMELSSLRSEDTAVYYCSRGELGGFAYWGQGTLVTVSS

SEQ ID NO: 426 - protein, 117 aa, synthetic construct
  REGION 1..117: note = Synthetic peptide
QVQLVQSGAEVKKPGASVKMSCKASGYTFTSYTMHWIRQAPGQGLEWIGYINPSSTYTHYIKKFKDRATLTADKSTSTAYMELSSLRSEDTAVYYCSRGELGGFAYWGQGTLVTVSS

SEQ ID NO: 427 - protein, 117 aa, synthetic construct
  REGION 1..117: note = Synthetic peptide
QVQLVQSGAEVKKPGASVKMSCKASGYTFTSYTMHWIRQAPGQGQEWIGYINPSSTYTHYIKKFKDRATLTADKSTSTAYMELSSLRSEDTAVYYCSRGELGGFAYWGQGTLVTVSS

SEQ ID NO: 428 - protein, 116 aa, synthetic construct
  REGION 1..116: note = Synthetic peptide
  VARIANT 5: note = Xaa can be any naturally occurring amino acid
  VARIANT 8: note = Xaa can be any naturally occurring amino acid
  VARIANT 11..13: note = Xaa can be any naturally occurring amino acid
  VARIANT 20: note = Xaa can be any naturally occurring amino acid
  VARIANT 31: note = Xaa can be any naturally occurring amino acid
  VARIANT 33: note = Xaa can be any naturally occurring amino acid
  VARIANT 35: note = Xaa can be any naturally occurring amino acid
  VARIANT 38: note = Xaa can be any naturally occurring amino acid
  VARIANT 40: note = Xaa can be any naturally occurring amino acid
  VARIANT 48: note = Xaa can be any naturally occurring amino acid
  VARIANT 50: note = Xaa can be any naturally occurring amino acid
  VARIANT 55: note = Xaa can be any naturally occurring amino acid
  VARIANT 57: note = Xaa can be any naturally occurring amino acid
  VARIANT 59: note = Xaa can be any naturally occurring amino acid
  VARIANT 61: note = Xaa can be any naturally occurring amino acid
  VARIANT 65..68: note = Xaa can be any naturally occurring amino acid
  VARIANT 70: note = Xaa can be any naturally occurring amino acid
  VARIANT 72: note = Xaa can be any naturally occurring amino acid
  VARIANT 74..76: note = Xaa can be any naturally occurring amino acid
  VARIANT 79..80: note = Xaa can be any naturally occurring amino acid
  VARIANT 82: note = Xaa can be any naturally occurring amino acid
  VARIANT 87: note = Xaa can be any naturally occurring amino acid
  VARIANT 90..91: note = Xaa can be any naturally occurring amino acid
  VARIANT 98: note = Xaa can be any naturally occurring amino acid
  VARIANT 101: note = Xaa can be any naturally occurring amino acid
  VARIANT 116: note = Xaa can be any naturally occurring amino acid
QVQLXQSXAEXXXPGASVKXSCKASGYTFTXYXMXWVXQXPGQGLEWXGXINPSXGXTXYXQKFXXXXTXTXDXSXSTXXMXLSSLXSEXXAVYYCAXGDXYVAYWGQGTLVTVSX

SEQ ID NO: 429 - protein, 116 aa, synthetic construct
  REGION 1..116: note = Synthetic peptide
  VARIANT 20: note = Xaa can be any naturally occurring amino acid
  VARIANT 31: note = Xaa can be any naturally occurring amino acid
  VARIANT 35: note = Xaa can be any naturally occurring amino acid
  VARIANT 48: note = Xaa can be any naturally occurring amino acid
  VARIANT 50: note = Xaa can be any naturally occurring amino acid
  VARIANT 59: note = Xaa can be any naturally occurring amino acid
  VARIANT 67: note = Xaa can be any naturally occurring amino acid
  VARIANT 70: note = Xaa can be any naturally occurring amino acid
  VARIANT 74: note = Xaa can be any naturally occurring amino acid
  VARIANT 79: note = Xaa can be any naturally occurring amino acid
  VARIANT 98: note = Xaa can be any naturally occurring amino acid
  VARIANT 101: note = Xaa can be any naturally occurring amino acid
QVQLVQSGAEVKKPGASVKXSCKASGYTFTXYTMXWVRQAPGQGLEWXGXINPSSGYTXYAQKFQGXVTXTADXSTSTXYMELSSLRSEDTAVYYCAXGDXYVAYWGQGTLVTVSS

SEQ ID NO: 430 - protein, 108 aa, synthetic construct
  REGION 1..108: note = Synthetic peptide
  VARIANT 1: note = Xaa can be any naturally occurring amino acid
  VARIANT 3..4: note = Xaa can be any naturally occurring amino acid
  VARIANT 9..11: note = Xaa can be any naturally occurring amino acid
  VARIANT 15: note = Xaa can be any naturally occurring amino acid
  VARIANT 17: note = Xaa can be any naturally occurring amino acid
  VARIANT 21: note = Xaa can be any naturally occurring amino acid
  VARIANT 24: note = Xaa can be any naturally occurring amino acid
  VARIANT 27: note = Xaa can be any naturally occurring amino acid
  VARIANT 29: note = Xaa can be any naturally occurring amino acid
  VARIANT 32: note = Xaa can be any naturally occurring amino acid
  VARIANT 34..35: note = Xaa can be any naturally occurring amino acid
  VARIANT 43..44: note = Xaa can be any naturally occurring amino acid
  VARIANT 48: note = Xaa can be any naturally occurring amino acid
  VARIANT 51..56: note = Xaa can be any naturally occurring amino acid
  VARIANT 61: note = Xaa can be any naturally occurring amino acid
  VARIANT 67: note = Xaa can be any naturally occurring amino acid
  VARIANT 71..73: note = Xaa can be any naturally occurring amino acid
  VARIANT 79..81: note = Xaa can be any naturally occurring amino acid
  VARIANT 84: note = Xaa can be any naturally occurring amino acid
  VARIANT 90..91: note = Xaa can be any naturally occurring amino acid
  VARIANT 93..96: note = Xaa can be any naturally occurring amino acid
  VARIANT 101: note = Xaa can be any naturally occurring amino acid
  VARIANT 107: note = Xaa can be any naturally occurring amino acid
XIXXTQSPXXXSASXGXRVTXTCXASXSXSSXYXXWYQQKPGXXPKLXIYXXXXXXSGVPXRFSGSXSGTXXXLTISSXXXEDXATYYCXXYXXXXLTFGXGTKLEXK

SEQ ID NO: 431 - protein, 108 aa, synthetic construct
  REGION 1..108: note = Synthetic peptide
  VARIANT 4: note = Xaa can be any naturally occurring amino acid
  VARIANT 21: note = Xaa can be any naturally occurring amino acid
  VARIANT 32: note = Xaa can be any naturally occurring amino acid
  VARIANT 34: note = Xaa can be any naturally occurring amino acid
  VARIANT 48: note = Xaa can be any naturally occurring amino acid
  VARIANT 51: note = Xaa can be any naturally occurring amino acid
  VARIANT 53: note = Xaa can be any naturally occurring amino acid
  VARIANT 61: note = Xaa can be any naturally occurring amino acid
  VARIANT 67: note = Xaa can be any naturally occurring amino acid
  VARIANT 79: note = Xaa can be any naturally occurring amino acid
  VARIANT 84: note = Xaa can be any naturally occurring amino acid
  VARIANT 91: note = Xaa can be any naturally occurring amino acid
  VARIANT 93: note = Xaa can be any naturally occurring amino acid
DIQXTQSPSSLSASVGDRVTXTCTASSSVSSXYXHWYQQKPGKAPKLXIYXTXNLASGVPXRFSGSXSGTDYTLTISSXQPEDXATYYCHXYXRSPLTFGQGTKLEIK

SEQ ID NO: 432 - protein, 117 aa, synthetic construct
  REGION 1..117: note = Synthetic peptide
  VARIANT 3: note = Xaa can be any naturally occurring amino acid
  VARIANT 5: note = Xaa can be any naturally occurring amino acid
  VARIANT 18..19: note = Xaa can be any naturally occurring amino acid
  VARIANT 23: note = Xaa can be any naturally occurring amino acid
  VARIANT 31: note = Xaa can be any naturally occurring amino acid
  VARIANT 33: note = Xaa can be any naturally occurring amino acid
  VARIANT 35: note = Xaa can be any naturally occurring amino acid
  VARIANT 40: note = Xaa can be any naturally occurring amino acid
  VARIANT 42: note = Xaa can be any naturally occurring amino acid
  VARIANT 49..50: note = Xaa can be any naturally occurring amino acid
  VARIANT 52..59: note = Xaa can be any naturally occurring amino acid
  VARIANT 61: note = Xaa can be any naturally occurring amino acid
  VARIANT 64: note = Xaa can be any naturally occurring amino acid
  VARIANT 76: note = Xaa can be any naturally occurring amino acid
  VARIANT 79..81: note = Xaa can be any naturally occurring amino acid
  VARIANT 87: note = Xaa can be any naturally occurring amino acid
  VARIANT 94..95: note = Xaa can be any naturally occurring amino acid
  VARIANT 99: note = Xaa can be any naturally occurring amino acid
  VARIANT 106: note = Xaa can be any naturally occurring amino acid
  VARIANT 112: note = Xaa can be any naturally occurring amino acid
  VARIANT 114: note = Xaa can be any naturally occurring amino acid
EVXLXESGGGLVQPGGSXXLSCXASGFTFSXYXMXWVRQXPXKGLEWVXXIXXXXXXXXTXYAXSVKGRFTISRDXSKXXXYLQMNXLRAEDTXXYYCXDGPPSGXWGQGTXLXVSS

SEQ ID NO: 433 - protein, 117 aa, synthetic construct
  REGION 1..117: note = Synthetic peptide
  VARIANT 31: note = Xaa can be any naturally occurring amino acid
  VARIANT 35: note = Xaa can be any naturally occurring amino acid
  VARIANT 50: note = Xaa can be any naturally occurring amino acid
  VARIANT 55: note = Xaa can be any naturally occurring amino acid
  VARIANT 79: note = Xaa can be any naturally occurring amino acid
  VARIANT 99: note = Xaa can be any naturally occurring amino acid
  VARIANT 106: note = Xaa can be any naturally occurring amino acid
EVQLLESGGGLVQPGGSMRLSCAASGFTFSXYWMXWVRQAPGKGLEWVAXIRLKXDNYATHYADSVKGRFTISRDDSKXTVYLQMNSLRAEDTGVYYCXDGPPSGXWGQGTLLTVSS

SEQ ID NO: 434 - protein, 107 aa, synthetic construct
  REGION 1..107: note = Synthetic peptide
  VARIANT 9: note = Xaa can be any naturally occurring amino acid
  VARIANT 17..18: note = Xaa can be any naturally occurring amino acid
  VARIANT 25: note = Xaa can be any naturally occurring amino acid
  VARIANT 27..28: note = Xaa can be any naturally occurring amino acid
  VARIANT 30: note = Xaa can be any naturally occurring amino acid
  VARIANT 34: note = Xaa can be any naturally occurring amino acid
  VARIANT 40: note = Xaa can be any naturally occurring amino acid
  VARIANT 43: note = Xaa can be any naturally occurring amino acid
  VARIANT 45: note = Xaa can be any naturally occurring amino acid
  VARIANT 48: note = Xaa can be any naturally occurring amino acid
  VARIANT 50: note = Xaa can be any naturally occurring amino acid
  VARIANT 52..53: note = Xaa can be any naturally occurring amino acid
  VARIANT 55..56: note = Xaa can be any naturally occurring amino acid
  VARIANT 70: note = Xaa can be any naturally occurring amino acid
  VARIANT 72: note = Xaa can be any naturally occurring amino acid
  VARIANT 74: note = Xaa can be any naturally occurring amino acid
  VARIANT 76: note = Xaa can be any naturally occurring amino acid
  VARIANT 84..85: note = Xaa can be any naturally occurring amino acid
  VARIANT 90..91: note = Xaa can be any naturally occurring amino acid
  VARIANT 93..94: note = Xaa can be any naturally occurring amino acid
  VARIANT 97: note = Xaa can be any naturally occurring amino acid
  VARIANT 100: note = Xaa can be any naturally occurring amino acid
DIQMTQSPXSLSASVGXXVTITCRXSXXIXSYLXWYQQKXGKXPXLLXYXAXXLXXGVPSRFSGSGSGTXFXLXIXSLQPEDFXXYYCQXXYXXPWXFGXGTKLEIK

SEQ ID NO: 435 - protein, 107 aa, synthetic construct
  REGION 1..107: note = Synthetic peptide
  VARIANT 25: note = Xaa can be any naturally occurring amino acid
  VARIANT 34: note = Xaa can be any naturally occurring amino acid
  VARIANT 48: note = Xaa can be any naturally occurring amino acid
  VARIANT 53: note = Xaa can be any naturally occurring amino acid
  VARIANT 55: note = Xaa can be any naturally occurring amino acid
  VARIANT 84..85: note = Xaa can be any naturally occurring amino acid
  VARIANT 90: note = Xaa can be any naturally occurring amino acid
  VARIANT 93: note = Xaa can be any naturally occurring amino acid
DIQMTQSPSSLSASVGDRVTITCRXSENIYSYLXWYQQKPGKAPKLLXYNAKXLXEGVPSRFSGSGSGTDFTLTISSLQPEDFXXYYCQXHYXVPWTFGQGTKLEIK

SEQ ID NO: 436 - protein, 117 aa, synthetic construct
  REGION 1..117: note = Synthetic peptide
  VARIANT 5: note = Xaa can be any naturally occurring amino acid
  VARIANT 11..13: note = Xaa can be any naturally occurring amino acid
  VARIANT 20: note = Xaa can be any naturally occurring amino acid
  VARIANT 29: note = Xaa can be any naturally occurring amino acid
  VARIANT 31: note = Xaa can be any naturally occurring amino acid
  VARIANT 33: note = Xaa can be any naturally occurring amino acid
  VARIANT 37..38: note = Xaa can be any naturally occurring amino acid
  VARIANT 40: note = Xaa can be any naturally occurring amino acid
  VARIANT 45: note = Xaa can be any naturally occurring amino acid
  VARIANT 48: note = Xaa can be any naturally occurring amino acid
  VARIANT 50: note = Xaa can be any naturally occurring amino acid
  VARIANT 55..57: note = Xaa can be any naturally occurring amino acid
  VARIANT 59: note = Xaa can be any naturally occurring amino acid
  VARIANT 61..62: note = Xaa can be any naturally occurring amino acid
  VARIANT 65..68: note = Xaa can be any naturally occurring amino acid
  VARIANT 70: note = Xaa can be any naturally occurring amino acid
  VARIANT 72: note = Xaa can be any naturally occurring amino acid
  VARIANT 74: note = Xaa can be any naturally occurring amino acid
  VARIANT 76: note = Xaa can be any naturally occurring amino acid
  VARIANT 79: note = Xaa can be any naturally occurring amino acid
  VARIANT 82: note = Xaa can be any naturally occurring amino acid
  VARIANT 84: note = Xaa can be any naturally occurring amino acid
  VARIANT 87: note = Xaa can be any naturally occurring amino acid
  VARIANT 91: note = Xaa can be any naturally occurring amino acid
  VARIANT 97: note = Xaa can be any naturally occurring amino acid
  VARIANT 101: note = Xaa can be any naturally occurring amino acid
  VARIANT 117: note = Xaa can be any naturally occurring amino acid
QVQLXQSGAEXXXPGASVKXSCKASGYTXTXYXMHWXXQXPGQGXEWXGXINPSXXXTXYXXKFXXXXTXTXDXSXSTXYMXLXSLXSEDXAVYYCXRGEXGGFAYWGQGTLVTVSX

SEQ ID NO: 437 - protein, 117 aa, synthetic construct
  REGION 1..117: note = Synthetic peptide
  VARIANT 20: note = Xaa can be any naturally occurring amino acid
  VARIANT 29: note = Xaa can be any naturally occurring amino acid
  VARIANT 31: note = Xaa can be any naturally occurring amino acid
  VARIANT 37: note = Xaa can be any naturally occurring amino acid
  VARIANT 45: note = Xaa can be any naturally occurring amino acid
  VARIANT 48: note = Xaa can be any naturally occurring amino acid
  VARIANT 56: note = Xaa can be any naturally occurring amino acid
  VARIANT 59: note = Xaa can be any naturally occurring amino acid
  VARIANT 61..62: note = Xaa can be any naturally occurring amino acid
  VARIANT 65..66: note = Xaa can be any naturally occurring amino acid
  VARIANT 68: note = Xaa can be any naturally occurring amino acid
  VARIANT 70: note = Xaa can be any naturally occurring amino acid
  VARIANT 74: note = Xaa can be any naturally occurring amino acid
  VARIANT 79: note = Xaa can be any naturally occurring amino acid
  VARIANT 84: note = Xaa can be any naturally occurring amino acid
  VARIANT 97: note = Xaa can be any naturally occurring amino acid
  VARIANT 101: note = Xaa can be any naturally occurring amino acid
QVQLVQSGAEVKKPGASVKXSCKASGYTXTXYTMHWXRQAPGQGXEWXGYINPSSXYTXYXXKFXXRXTXTADXSTSTXYMELXSLRSEDTAVYYCXRGEXGGFAYWGQGTLVTVSS

SEQ ID NO: 438 - protein, 112 aa, synthetic construct
  REGION 1..112: note = Synthetic peptide
  VARIANT 7: note = Xaa can be any naturally occurring amino acid
  VARIANT 14: note = Xaa can be any naturally occurring amino acid
  VARIANT 17..18: note = Xaa can be any naturally occurring amino acid
  VARIANT 31: note = Xaa can be any naturally occurring amino acid
  VARIANT 33: note = Xaa can be any naturally occurring amino acid
  VARIANT 39: note = Xaa can be any naturally occurring amino acid
  VARIANT 41..42: note = Xaa can be any naturally occurring amino acid
  VARIANT 44: note = Xaa can be any naturally occurring amino acid
  VARIANT 50..51: note = Xaa can be any naturally occurring amino acid
  VARIANT 55: note = Xaa can be any naturally occurring amino acid
  VARIANT 57: note = Xaa can be any naturally occurring amino acid
  VARIANT 81: note = Xaa can be any naturally occurring amino acid
  VARIANT 88: note = Xaa can be any naturally occurring amino acid
  VARIANT 92: note = Xaa can be any naturally occurring amino acid
  VARIANT 94..96: note = Xaa can be any naturally occurring amino acid
  VARIANT 99..100: note = Xaa can be any naturally occurring amino acid
  VARIANT 105: note = Xaa can be any naturally occurring amino acid
DVVMTQXPLSLPVXLGXXASISCRSSQSLVXSXGNTYLXWXXQXPGQSPXXNPSXTXTHYSGVPDRFSGSGSGTDFTLKIXRVEAEDXGVYXCXXXTHXXYTFGXGTKLEIK

SEQ ID NO: 439 - protein, 112 aa, synthetic construct
  REGION 1..112: note = Synthetic peptide
  VARIANT 33: note = Xaa can be any naturally occurring amino acid
  VARIANT 39: note = Xaa can be any naturally occurring amino acid
  VARIANT 55: note = Xaa can be any naturally occurring amino acid
  VARIANT 57: note = Xaa can be any naturally occurring amino acid
  VARIANT 81: note = Xaa can be any naturally occurring amino acid
  VARIANT 95..96: note = Xaa can be any naturally occurring amino acid
DVVMTQSPLSLPVTLGQPASISCRSSQSLVHSXGNTYLXWYQQRPGQSPRLLIYXVXNRFSGVPDRFSGSGSGTDFTLKIXRVEAEDVGVYYCSXXTHVPYTFGQGTKLEIK

SEQ ID NO: 440 - protein, 120 aa, synthetic construct
  REGION 1..120: note = Synthetic peptide
  VARIANT 5: note = Xaa can be any naturally occurring amino acid
  VARIANT 9: note = Xaa can be any naturally occurring amino acid
  VARIANT 11..12: note = Xaa can be any naturally occurring amino acid
  VARIANT 20: note = Xaa can be any naturally occurring amino acid
  VARIANT 38: note = Xaa can be any naturally occurring amino acid
  VARIANT 40..41: note = Xaa can be any naturally occurring amino acid
  VARIANT 43..44: note = Xaa can be any naturally occurring amino acid
  VARIANT 48: note = Xaa can be any naturally occurring amino acid
  VARIANT 61: note = Xaa can be any naturally occurring amino acid
  VARIANT 65: note = Xaa can be any naturally occurring amino acid
  VARIANT 67..68: note = Xaa can be any naturally occurring amino acid
  VARIANT 70: note = Xaa can be any naturally occurring amino acid
  VARIANT 72: note = Xaa can be any naturally occurring amino acid
  VARIANT 74: note = Xaa can be any naturally occurring amino acid
  VARIANT 76: note = Xaa can be any naturally occurring amino acid
  VARIANT 79: note = Xaa can be any naturally occurring amino acid
  VARIANT 82: note = Xaa can be any naturally occurring amino acid
  VARIANT 84: note = Xaa can be any naturally occurring amino acid
  VARIANT 87: note = Xaa can be any naturally occurring amino acid
  VARIANT 91: note = Xaa can be any naturally occurring amino acid
  VARIANT 116: note = Xaa can be any naturally occurring amino acid
QVQLXQSGXEXXKPGASVKXSCKASGYSFTGYNMNWVXQXXGXXLEWXGNIDPYYGGSTYXQKFXGXXTXTXDXSXSTXYMXLXSLXSEDXAVYYCARERSGYVFSAMDYWGQGTXVTVS

SEQ ID NO: 441 - protein, 120 aa, synthetic construct
  REGION 1..120: note = Synthetic peptide
  VARIANT 20: note = Xaa can be any naturally occurring amino acid
  VARIANT 48: note = Xaa can be any naturally occurring amino acid
  VARIANT 68: note = Xaa can be any naturally occurring amino acid
  VARIANT 70: note = Xaa can be any naturally occurring amino acid
  VARIANT 79: note = Xaa can be any naturally occurring amino acid
QVQLVQSGAEVKKPGASVKXSCKASGYSFTGYNMNWVRQAPGQGLEWXGNIDPYYGGSTYAQKFQGRXTXTRDTSTSTXYMELSSLRSEDTAVYYCARERSGYVFSAMDYWGQGTLVTVS

SEQ ID NO: 442 - protein, 112 aa, synthetic construct
  REGION 1..112: note = Synthetic peptide
  VARIANT 1: note = Xaa can be any naturally occurring amino acid
  VARIANT 3: note = Xaa can be any naturally occurring amino acid
  VARIANT 9: note = Xaa can be any naturally occurring amino acid
  VARIANT 15: note = Xaa can be any naturally occurring amino acid
  VARIANT 18..19: note = Xaa can be any naturally occurring amino acid
  VARIANT 21..22: note = Xaa can be any naturally occurring amino acid
  VARIANT 49: note = Xaa can be any naturally occurring amino acid
  VARIANT 51: note = Xaa can be any naturally occurring amino acid
  VARIANT 69: note = Xaa can be any naturally occurring amino acid
  VARIANT 78: note = Xaa can be any naturally occurring amino acid
  VARIANT 84: note = Xaa can be any naturally occurring amino acid
  VARIANT 93: note = Xaa can be any naturally occurring amino acid
  VARIANT 105: note = Xaa can be any naturally occurring amino acid
  VARIANT 111: note = Xaa can be any naturally occurring amino acid
XIXMTQSPXSLAVSXGEXXTXXCKSSQSVLFSSNQKNYLAWYQQKPGQXPXLLIYWASTRESGVPDRFXGSGSGTDFXLTISSXQAEDVAVYXCHQYLSSRTFGXGTKLEXK

SEQ ID NO: 443 - protein, 112 aa, synthetic construct
  REGION 1..112: note = Synthetic peptide
  VARIANT 19: note = Xaa can be any naturally occurring amino acid
  VARIANT 21: note = Xaa can be any naturally occurring amino acid
  VARIANT 84: note = Xaa can be any naturally occurring amino acid
DIVMTQSPDSLAVSLGERXTXNCKSSQSVLFSSNQKNYLAWYQQKPGQPPKLLIYWASTRESGVPDRFSGSGSGTDFTLTISSXQAEDVAVYYCHQYLSSRTFGQGTKLEIK

SEQ ID NO: 444 - protein, 117 aa, synthetic construct
  REGION 1..117: note = Synthetic peptide
  VARIANT 1: note = Xaa can be any naturally occurring amino acid
  VARIANT 5: note = Xaa can be any naturally occurring amino acid
  VARIANT 9: note = Xaa can be any naturally occurring amino acid
  VARIANT 11..12: note = Xaa can be any naturally occurring amino acid
  VARIANT 20: note = Xaa can be any naturally occurring amino acid
  VARIANT 38: note = Xaa can be any naturally occurring amino acid
  VARIANT 40..41: note = Xaa can be any naturally occurring amino acid
  VARIANT 43..44: note = Xaa can be any naturally occurring amino acid
  VARIANT 48: note = Xaa can be any naturally occurring amino acid
  VARIANT 61: note = Xaa can be any naturally occurring amino acid
  VARIANT 63: note = Xaa can be any naturally occurring amino acid
  VARIANT 65: note = Xaa can be any naturally occurring amino acid
  VARIANT 67: note = Xaa can be any naturally occurring amino acid
  VARIANT 69..70: note = Xaa can be any naturally occurring amino acid
  VARIANT 72..74: note = Xaa can be any naturally occurring amino acid
  VARIANT 76: note = Xaa can be any naturally occurring amino acid
  VARIANT 79: note = Xaa can be any naturally occurring amino acid
  VARIANT 84: note = Xaa can be any naturally occurring amino acid
  VARIANT 87: note = Xaa can be any naturally occurring amino acid
  VARIANT 91: note = Xaa can be any naturally occurring amino acid
  VARIANT 93: note = Xaa can be any naturally occurring amino acid
  VARIANT 112..113: note = Xaa can be any naturally occurring amino acid
XVQLXQSGXEXXKPGASVKXSCKASGYRFTDYNMHWVXQXXGXXLEWXGYINPNNGGTNYXQXFXGXVXXTXXXSXSTXYMELXSLXSEDXAXYYCARDYLYFFDCWGQGTXXTVSS

SEQ ID NO: 445 - protein, 107 aa, synthetic construct
  REGION 1..107: note = Synthetic peptide
  VARIANT 9: note = Xaa can be any naturally occurring amino acid
  VARIANT 11: note = Xaa can be any naturally occurring amino acid
  VARIANT 15: note = Xaa can be any naturally occurring amino acid
  VARIANT 17..18: note = Xaa can be any naturally occurring amino acid
  VARIANT 43: note = Xaa can be any naturally occurring amino acid
  VARIANT 45: note = Xaa can be any naturally occurring amino acid
  VARIANT 70: note = Xaa can be any naturally occurring amino acid
  VARIANT 72..74: note = Xaa can be any naturally occurring amino acid
  VARIANT 80: note = Xaa can be any naturally occurring amino acid
  VARIANT 84..85: note = Xaa can be any naturally occurring amino acid
  VARIANT 100: note = Xaa can be any naturally occurring amino acid
DIQMTQSPXSXSASXGXXVTITCLASQTIGTWLAWYQQKPGKXPXLLIYAAASLADGVPSRFSGSGSGTXFXXXISSLQXEDFXXYYCQQLYSIPRTFGXGTKLEIK

SEQ ID NO: 446 - protein, 107 aa, synthetic construct
  REGION 1..107: note = Synthetic peptide
  VARIANT 1: note = Xaa can be any naturally occurring amino acid
  VARIANT 15: note = Xaa can be any naturally occurring amino acid
  VARIANT 18..19: note = Xaa can be any naturally occurring amino acid
  VARIANT 42: note = Xaa can be any naturally occurring amino acid
  VARIANT 49: note = Xaa can be any naturally occurring amino acid
  VARIANT 63: note = Xaa can be any naturally occurring amino acid
  VARIANT 75..76: note = Xaa can be any naturally occurring amino acid
  VARIANT 78: note = Xaa can be any naturally occurring amino acid
  VARIANT 80: note = Xaa can be any naturally occurring amino acid
  VARIANT 84: note = Xaa can be any naturally occurring amino acid
  VARIANT 88: note = Xaa can be any naturally occurring amino acid
  VARIANT 93: note = Xaa can be any naturally occurring amino acid
XVQLVESGGGLVQPXGSXXLSCAASGFTFSSFGMHWVRQAPXKGLEWVXYISSDSRTIYYADXVKGRFTISRDNXXNXLXLQMXSLRXEDTAXYYCARDYGRTYEAY

SEQ ID NO: 447 - protein, 111 aa, synthetic construct
  REGION 1..111: note = Synthetic peptide
  VARIANT 4: note = Xaa can be any naturally occurring amino acid
  VARIANT 9: note = Xaa can be any naturally occurring amino acid
  VARIANT 17: note = Xaa can be any naturally occurring amino acid
  VARIANT 22: note = Xaa can be any naturally occurring amino acid
  VARIANT 64: note = Xaa can be any naturally occurring amino acid
  VARIANT 78: note = Xaa can be any naturally occurring amino acid
  VARIANT 80..84: note = Xaa can be any naturally occurring amino acid
  VARIANT 87: note = Xaa can be any naturally occurring amino acid
  VARIANT 89: note = Xaa can be any naturally occurring amino acid
  VARIANT 104: note = Xaa can be any naturally occurring amino acid
  VARIANT 110: note = Xaa can be any naturally occurring amino acid
DIVXTQSPXSLAVSLGXRATIXCRASKSVSTSGYSYIHWYQQKPGQPPKLLIYLASNLESGVPXRFSGSGSGTDFTLXIXXXXXEDXAXYYCQHSRELPLTFGXGTKLEXK

SEQ ID NO: 448 - protein, 111 aa, synthetic construct
  REGION 1..111: note = Synthetic peptide
  VARIANT 4: note = Xaa can be any naturally occurring amino acid
  VARIANT 82: note = Xaa can be any naturally occurring amino acid
  VARIANT 110: note = Xaa can be any naturally occurring amino acid
DIVXTQSPDSLAVSLGERATINCRASKSVSTSGYSYIHWYQQKPGQPPKLLIYLASNLESGVPDRFSGSGSGTDFTLTISSXQAEDVAVYYCQHSRELPLTFGQGTKLEXK

SEQ ID NO: 449 - protein, 7 aa, synthetic construct
  REGION 1..7: note = Synthetic peptide
  VARIANT 6: note = Xaa is T, V, F, or D
SSVSSXY

SEQ ID NO: 450 - skipped

SEQ ID NO: 451 - protein, 9 aa, synthetic construct
  REGION 1..9: note = Synthetic peptide
  VARIANT 2: note = Xaa is Q, H or S
  VARIANT 4: note = Xaa is H, Y, Q, or S
HXYXRSPLT

SEQ ID NO: 452 - protein, 7 aa, synthetic construct
  REGION 1..7: note = Synthetic peptide
  VARIANT 5: note = Xaa is T, V, D, or S
YTFTXYT

SEQ ID NO: 453 - protein, 9 aa, synthetic construct
  REGION 1..9: note = Synthetic peptide
  VARIANT 2: note = Xaa is N, Q, H, D, S, R, or A
AXGDYYVAY

SEQ ID NO: 454 - protein, 9 aa, synthetic construct
  REGION 1..9: note = Synthetic peptide
  VARIANT 2: note = Xaa is H, Q, S, or T
  VARIANT 5: note = Xaa is T, S, N, or G
QXHYXVPWT

SEQ ID NO: 455 - protein, 7 aa, synthetic construct
  REGION 1..7: note = Synthetic peptide
  VARIANT 5: note = Xaa is N, S, R, q, s, or a
  VARIANT 7: note = Xaa is w, h, y, or f
FTFSXYX

SEQ ID NO: 456 - protein, 10 aa, synthetic construct
  REGION 1..10: note = Synthetic peptide
  VARIANT 5: note = Xaa is S, N, A, or T
  VARIANT 7: note = Xaa is Q, S,A, or N
IRLKXDXYAT

SEQ ID NO: 457 - protein, 8 aa, synthetic construct
  REGION 1..8: note = Synthetic peptide
  VARIANT 1: note = Xaa is N, D, A, or T
  VARIANT 8: note = Xaa is S, T, A, C, Y
XDGPPSGX

SEQ ID NO: 458 - protein, 11 aa, synthetic construct
  REGION 1..11: note = Synthetic peptide
  VARIANT 7: note = Xaa is D, N, E, Q, S, or A
  VARIANT 9: note = Xaa is Q, S, A, D, or N
QSLVHSXGXTY

SEQ ID NO: 459 - skipped

SEQ ID NO: 460 - protein, 9 aa, synthetic construct
  REGION 1..9: note = Synthetic peptide
  VARIANT 2: note = Xaa is Q, H, or T
  VARIANT 3: note = Xaa is S, G, T, or D
SXXTHVPYT

SEQ ID NO: 461 - protein, 9 aa, synthetic construct
  REGION 1..9: note = Synthetic peptide
  VARIANT 3: note = Xaa is F, Y, S, or T
  VARIANT 5: note = Xaa is S, T, Y , or D
YTXTXYTMH

SEQ ID NO: 462 - protein, 8 aa, synthetic construct
  REGION 1..8: note = Synthetic peptide
  VARIANT 2: note = Xaa is Q, S, A, or N
  VARIANT 6: note = Xaa is T, S, V, D, or G
IXPSSXYT

SEQ ID NO: 463 - protein, 10 aa, synthetic construct
  REGION 1..10: note = Synthetic peptide
  VARIANT 1: note = Xaa is S, A, T, or V
  VARIANT 5: note = Xaa is L, V, or F
XRGEXGGFAY

SEQ ID NO: 464 - protein, 6 aa, synthetic construct
  REGION 1..6: note = Synthetic peptide
  VARIANT 6: note = Xaa is W, H, Y, or F
QTIGYX

SEQ ID NO: 465 - protein, 8 aa, synthetic construct
  REGION 1..8: note = Synthetic peptide
  VARIANT 3: note = Xaa is R or T
  VARIANT 8: note = Xaa is N, Q, S, or A
GYXFTDYX

SEQ ID NO: 466 - protein, 8 aa, synthetic construct
  REGION 1..8: note = Synthetic peptide
  VARIANT 2: note = Xaa is N, Q, S, or A
  VARIANT 4: note = Xaa is N, Q, S, or A
  VARIANT 5: note = Xaa is N, Q, S, or A
IXPXXGGT

SEQ ID NO: 467 - protein, 8 aa, synthetic construct
  REGION 1..8: note = Synthetic peptide
  VARIANT 8: note = Xaa is C, Y, S, or A
DYLYFFDX

SEQ ID NO: 468 - protein, 8 aa, synthetic construct
  REGION 1..8: note = Synthetic peptide
  VARIANT 4: note = Xaa is D, E, S, or A
ISSXSRTI

SEQ ID NO: 469 - protein, 9 aa, synthetic construct
  REGION 1..9: note = Synthetic peptide
DYGRTYEAY

SEQ ID NO: 470 - protein, 12 aa, synthetic construct
  REGION 1..12: note = Synthetic peptide
  VARIANT 8: note = Xaa is Q, S, A, D, or N
  VARIANT 11: note = Xaa is Q, S, A, D, or N
QSVLFSSXQKXY

SEQ ID NO: 471 - skipped

SEQ ID NO: 472 - protein, 8 aa, synthetic construct
  REGION 1..8: note = Synthetic peptide
  VARIANT 8: note = Xaa is N, Q, S, or A
GYSFTFYX

SEQ ID NO: 473 - protein, 8 aa, synthetic construct
  REGION 1..8: note = Synthetic peptide
  VARIANT 2: note = Xaa is A, S, E, or D
IXPYYGGS

SEQ ID NO: 474 - protein, 12 aa, synthetic construct
  REGION 1..12: note = Synthetic peptide
ERSGYVFSAMDY

SEQ ID NO: 475 - protein, 8 aa, synthetic construct
  REGION 1..8: note = Synthetic peptide
  VARIANT 2: note = Xaa is Q, S, A, or N
IXPSSGYT

SEQ ID NO: 476 - protein, 6 aa, synthetic construct
  REGION 1..6: note = Synthetic peptide
  VARIANT 2: note = Xaa is Q, S, A, D, or N
EXIYSY

SEQ ID NO: 477 - skipped

SEQ ID NO: 478 - protein, 116 aa, synthetic construct
  REGION 1..116: note = Synthetic peptide
  VARIANT 20: note = Xaa is M or V
  VARIANT 31: note = Xaa is T, V, D, or S
  VARIANT 48: note = Xaa is I or M
  VARIANT 52: note = Xaa is Q, S, A, or N
  VARIANT 70: note = Xaa is L or M
  VARIANT 74: note = Xaa is T or K
  VARIANT 98: note = Xaa is N, Q, H, D, S, R,or A
QVQLVQSGAEVKKPGASVKXSCKASGYTFTXYTMHWVRQAPGQGLEWXGFIXPSSGYTDYAQKFQGRVTXTADXSTSTVYMELSSLRSEDTAVYYCAXGDYYVAYWGQGTLVTVSS

SEQ ID NO: 479 - protein, 108 aa, synthetic construct
  REGION 1..108: note = Synthetic peptide
  VARIANT 4: note = Xaa is L or M
  VARIANT 21: note = Xaa is M or I
  VARIANT 32: note = Xaa is T, V, F, or D
  VARIANT 48: note = Xaa is W or L
  VARIANT 51: note = Xaa is S, t, Q or A
  VARIANT 53: note = Xaa is S,T, D or Q
  VARIANT 79: note = Xaa is M or L
  VARIANT 84: note = Xaa is A or F
  VARIANT 91: note = Xaa is Q, H or S
  VARIANT 93: note = Xaa is H, Y, Q, or S
DIQXTQSPSSLSASVGDRVTXTCTASSSVSSXYFHWYQQKPGKAPKLXIYXTXNLASGVPSRFSGSGSGTDYTLTISSXQPEDXATYYCHXYXRSPLTFGQGTKLEIK

SEQ ID NO: 480 - protein, 117 aa, synthetic construct
  REGION 1..117: note = Synthetic peptide
  VARIANT 31: note = Xaa is N, S, R, Q or A
  VARIANT 33: note = Xaa is W, H, Y or F
  VARIANT 55: note = Xaa is S, N, A, or T
  VARIANT 57: note = Xaa is Q, S, A, or N
  VARIANT 99: note = Xaa is N, D, or T
  VARIANT 106: note = Xaa is S, T, A, C, or Y
EVQLLESGGGLVQPGGSMRLSCAASGFTFSXYXMNWVRQAPGKGLEWVAQIRLKXDXYATHYADSVKGRFTISRDDSKNTVYLQMNSLRAEDTGVYYCXDGPPSGXWGQGTLLTVSS

SEQ ID NO: 481 - protein, 107 aa, synthetic construct
  REGION 1..107: note = Synthetic peptide
  VARIANT 28: note = Xaa is Q, S, A, D, or N
  VARIANT 48: note = Xaa is V or I
  VARIANT 50: note = Xaa is S, T, Q or A
  VARIANT 84: note = Xaa is G or A
  VARIANT 90: note = Xaa is H, Q, S or T
  VARIANT 93: note = Xaa is T, S, N, or G
DIQMTQSPSSLSASVGDRVTITCRISEXIYSYLAWYQQKPGKAPKLLXYXAKILVEGVPSRFSGSGSGTDFTLTISSLQPEDFXTYYCQXHYXVPWTFGQGTKLEIK

SEQ ID NO: 482 - protein, 117 aa, synthetic construct
  REGION 1..117: note = Synthetic peptide
  VARIANT 20: note = Xaa is M or V
  VARIANT 29: note = Xaa is F, Y, S or T
  VARIANT 31: note = Xaa is S, T, Y, or D
  VARIANT 37: note = Xaa is I or V
  VARIANT 45: note = Xaa is Q or L
  VARIANT 48: note = Xaa is I or M
  VARIANT 52: note = Xaa is Q, S, A, or N
  VARIANT 56: note = Xaa is T, S, V, D or G
  VARIANT 61: note = Xaa is I or A
  VARIANT 62: note = Xaa is K or Q
  VARIANT 65: note = Xaa is K or Q
  VARIANT 66: note = Xaa is D or G
  VARIANT 68: note = Xaa is A or V
  VARIANT 70: note = Xaa is L or M
  VARIANT 74: note = Xaa is T or K
  VARIANT 79: note = Xaa is A or V
  VARIANT 97: note = Xaa is S, A, T, or V
  VARIANT 101: note = Xaa is L, V, or F
QVQLVQSGAEVKKPGASVKXSCKASGYTXTXYTMHWXRQAPGQGXEWXGYIXPSSXYTHYXXKFXXRXTXTADXSTSTXYMELSSLRSEDTAVYYCXRGEXGGFAYWGQGTLVTVSS

SEQ ID NO: 483 - protein, 112 aa, synthetic construct
  REGION 1..112: note = Synthetic peptide
  VARIANT 33: note = Xaa is D, N, E, Q, S, or A
  VARIANT 35: note = Xaa is Q, S, A, D, or N
  VARIANT 55: note = Xaa is K, Q, or R
  VARIANT 57: note = Xaa is S, T, or V
  VARIANT 95: note = Xaa is Q, H, or T
  VARIANT 96: note = Xaa is S, G, T, or D
DVVMTQSPLSLPVTLGQPASISCRSSQSLVHSDGXTYLNWYQQRPGQSPRLLIYXVXNRFSGVPDRFSGSGSGTDFTLKISRVEAEDVGVYYCSXXTHVPYTFGQGTKLEIK

SEQ ID NO: 484 - protein, 121 aa, synthetic construct
  REGION 1..121: note = Synthetic peptide
  VARIANT 20: note = Xaa is I or V
  VARIANT 33: note = Xaa is N, Q, S, or A
  VARIANT 48: note = Xaa is I or M
  VARIANT 52: note = Xaa is A, S, E or D
  VARIANT 68: note = Xaa is A or V
  VARIANT 70: note = Xaa is L or M
  VARIANT 79: note = Xaa is A or V
QVQLVQSGAEVKKPGASVKXSCKASGYSFTGYXMNWVRQAPGQGLEWXGNIXPYYGGSTYAQKFQGRXTXTVDTSTSTXYMELSSLRSEDTAVYYCARERSGYVFSAMDYWGQGTLVTVSS

SEQ ID NO: 485 - protein, 112 aa, synthetic construct
  REGION 1..112: note = Synthetic peptide
  VARIANT 19: note = Xaa is V or A
  VARIANT 21: note = Xaa is M or I
  VARIANT 34: note = Xaa is Q, S, A, D, or N
  VARIANT 37: note = Xaa is Q, S, A, D, or N
  VARIANT 56: note = Xaa is H, Y, F, or W
  VARIANT 84: note = Xaa is V or L
DIVMTQSPDSLAVSLGERXTXNCKSSQSVLFSSXQKXYLAWYQQKPGQPPKLLIYXASTRESGVPDRFSGSGSGTDFTLTISSXQAEDVAVYYCHQYLSSRTFGQGTKLEIK

SEQ ID NO: 486 - protein, 118 aa, synthetic construct
  REGION 1..118: note = Synthetic peptide
  VARIANT 54: note = Xaa is D, E, S, or A
EVQLVESGGGLVQPGGSLRLSCAASGFTFSSFGMHWVRQAPGKGLEWVAYISSXSRTIYYADSVKGRFTISRDNAKNSLYLQMNSLRAEDTAVYYCARDYGRTYEAYWGQGTLVTVSS

SEQ ID NO: 487 - protein, 111 aa, synthetic construct
  REGION 1..111: note = Synthetic peptide
  VARIANT 4: note = Xaa is M or L
  VARIANT 82: note = Xaa is V or L
  VARIANT 110: note = Xaa is I or L
DIVXTQSPDSLAVSLGERATINCRASKSVSTSGYSYIHWYQQKPGQPPKLLIYLASNLESGVPDRFSGSGSGTDFTLTISSXQAEDVAVYYCQHSRELPLTFGQGTKLEIK

SEQ ID NO: 488 - protein, 117 aa, synthetic construct
  REGION 1..117: note = Synthetic peptide
  VARIANT 28: note = Xaa is R or T
  VARIANT 33: note = Xaa is N, Q, S or A
  VARIANT 52: note = Xaa is N, Q, S or A
  VARIANT 54: note = Xaa is N, Q, S or A
  VARIANT 55: note = Xaa is N, Q, S, or A
  VARIANT 106: note = Xaa is C, Y, S, or A
QVQLVQSGAEVKKPGASVKMSCKASGYXFTDYXMHWVRQAPGQGLEWIGYIXPXXGGTNYAQKFQGRATLTVDTSTSTAYMELSSLRSEDTAVYYCARDYLYFFDXWGQGTLLTVSS

SEQ ID NO: 489 - protein, 107 aa, synthetic construct
  REGION 1..107: note = Synthetic peptide
  VARIANT 24: note = Xaa is L or R
  VARIANT 32: note = Xaa is W, H, Y, or F
DIQMTQSPSSLSASVGDRVTITCLASQTIGTXLAWYQQKPGKAPKLLIYAAASLADGVPSRFSGSGSGTDFTFTISSLQPEDFVTYYCQQLYSIPRTFGQGTKLEIK